European Patent Specification EP 4 047 018 B1, published December 13, 2023. Title: TETRAVALENT BISPECIFIC ANTIBODY AGAINST PD-1 AND VEGF, PREPARATION METHOD THEREFOR, AND USE THEREOF. Applicant: SUNSHINE GUOJIAN PHARMACEUTICAL (SHANGHAI) CO., LTD. The sequence listing filed with the application follows.

SEQUENCE LISTING (153 sequences)

SEQ ID NO: 1 - protein, 123 aa, Homo [sequence omitted]

SEQ ID NO: 2 - protein, 107 aa, Homo [sequence omitted]

SEQ ID NO: 3 - protein, 118 aa, Mus musculus
EVKLVESGGGLVEPGGSLKLSCAASGFVFSNYDMSWVRQTPEKRLEWVATISGGGGYTYYSDSVKGRFTISRDNARNTLYLQMTSLRSEDTALFYCASPYGHYGFEYWGQGTTLTVSS

SEQ ID NO: 4 - protein, 107 aa, Mus musculus
DIQMTQTTSSLSASLGDRVTISCSASQGISNFLSWYQQKPDGTVKLLIYYTSSLHSGVPSRFSGSGSGTDYSLTISNLEPEDIATYYCQQYSNLPWTFGGGTKLEIR

SEQ ID NO: 5 - protein, 5 aa, Mus musculus
NYDMS

SEQ ID NO: 6 - protein, 17 aa, Mus musculus
TISGGGGYTYYSDSVKG

SEQ ID NO: 7 - protein, 9 aa, Mus musculus
PYGHYGFEY

SEQ ID NO: 8 - protein, 11 aa, Mus musculus
SASQGISNFLS

SEQ ID NO: 9 - protein, 7 aa, Mus musculus
YTSSLHS

SEQ ID NO: 10 - protein, 9 aa, Mus musculus
QQYSNLPWT

SEQ ID NO: 11 - protein, 118 aa, Homo
EVQLVESGGGLVQPGGSLRLSCAASGFVFSNYDMSWVRQAPGKRLEWVATISGGGGYTYYSDSVKGRFTISRDNAKNSLYLQMNSLRAEDTAVYYCASPYGHYGFEYWGQGTLVTVSS

SEQ ID NO: 12 - protein, 107 aa, Homo
DIQMTQSPSSLSASVGDRVTITCSASQGISNFLSWYQQKPGKTVKLLIYYTSSLHSGVPSRFSGSGSGTDYTFTISSLQPEDIATYYCQQYSNLPWTFGQGTKVEIK

SEQ ID NO: 13 - protein, 214 aa, Homo
DIQMTQSPSSLSASVGDRVTITCSASQDISNYLNWYQQKPGKAPKVLIYFTSSLHSGVPSRFSGSGSGTDFTLTISSLQPEDFATYYCQQYSTLPWTFGQGTKVEIKRTVAAPSVFIFPPSDEQLKSGTASVVCLLNNFYPREAKVQWKVDNALQSGNSQESVTEQDSKDSTYSLSSTLTLSKADYEKHKVYACEVTHQGLSSPVTKSFNRGEC

SEQ ID NO: 14 - DNA, 642 bp, Homo
gacatccagatgacccagtcccccagcagcctgagcgccagcgtgggcgacagggtgaccatcacctgctccgcctcccaggacatctccaactacctgaactggtaccagcagaagcccggcaaggcccccaaggtgctgatctacttcacctcctccctgcactccggcgtgcccagcaggttctccggcagcggctccggcaccgacttcaccctgaccatctccagcctgcagcccgaggacttcgccacctactactgccagcagtactccaccctgccctggaccttcggccagggcaccaaggtggagatcaagaggaccgtggccgccccctccgtgttcatcttccccccctccgacgagcagctgaagagcggcaccgccagcgtggtgtgcctgctgaacaacttctaccccagggaggccaaggtgcagtggaaggtggacaacgccctgcagagcggcaactcccaggagagcgtgaccgagcaggactccaaggactccacctacagcctgagctccaccctgaccctgtccaaggccgactacgagaagcacaaggtgtacgcctgcgaggtgacccaccagggcctgtcctcccccgtgaccaagtccttcaacaggggcgagtgc

SEQ ID NO: 15 - protein, 107 aa, Homo
DIQMTQSPSSLSASVGDRVTITCSASQDISNYLNWYQQKPGKAPKVLIYFTSSLHSGVPSRFSGSGSGTDFTLTISSLQPEDFATYYCQQYSTLPWTFGQGTKVEIK

SEQ ID NO: 16 - protein, 681 aa, Homo
EVQLVESGGGLVQPGGSLRLSCAASGFVFSNYDMSWVRQAPGKRLEWVATISGGGGYTYYSDSVKGRFTISRDNAKNSLYLQMNSLRAEDTAVYYCASPYGHYGFEYWGQGTLVTVSSASTKGPSVFPLAPCSRSTSESTAALGCLVKDYFPEPVTVSWNSGALTSGVHTFPAVLQSSGLYSLSSVVTVPSSSLGTKTYTCNVDHKPSNTKVDKRVGGGGSGGGGSGGGGSEVQLVESGGGLVQPGGSLRLSCAASGYTFTNYGMNWVRQAPGKGLEWVGWINTYTGEPTYAADFKRRFTFSLDTSKSTAYLQMNSLRAEDTAVYYCAKYPHYYGSSHWYFDVWGQGTLVTVSSASTKGPSVFPLAPCSRSTSESTAALGCLVKDYFPEPVTVSWNSGALTSGVHTFPAVLQSSGLYSLSSVVTVPSSSLGTKTYTCNVDHKPSNTKVDKRVESKYGPPCPPCPAPEFLGGPSVFLFPPKPKDTLMISRTPEVTCVVVDVSQEDPEVQFNWYVDGVEVHNAKTKPREEQFNSTYRVVSVLTVLHQDWLNGKEYKCKVSNKGLPSSIEKTISKAKGQPREPQVYTLPPSQEEMTKNQVSLTCLVKGFYPSDIAVEWESNGQPENNYKTTPPVLDSDGSFFLYSRLTVDKSRWQEGNVFSCSVMHEALHNHYTQKSLSLSLGK

SEQ ID NO: 17 - DNA, 2043 bp, Homo
gaggtccagctggtggagagcggaggaggactggtgcagcccggcggctctctgaggctgagctgtgccgctagcggcttcgtcttctccaactacgacatgagctgggtgaggcaagcccccggcaagaggctggagtgggtggctacaatcagcggcggcggaggctacacatactactccgactccgtgaagggaaggttcactatctctagggacaacgccaagaactctctgtatctgcagatgaactctctgagagccgaggatacagctgtgtactactgtgcctccccatacggccactacggcttcgagtactggggccaaggcactctggtcactgtgagcagcgcaagtaccaagggacctagtgttttccctcttgcaccttgctccaggtcaacatcagagtccacagctgctcttggatgtctcgttaaggactacttcccagagccagttaccgtatcctggaactccggagctttgacaagcggcgttcatacattcccagctgtgttgcagagttctgggttgtacagtttgagctcagtggtgaccgtgccttcatcttctttgggcactaagacctacacctgcaacgtggatcacaagccaagcaacaccaaggtggataagagggtgggtggaggcggttcaggcggaggtggcagcggaggtggcgggagtgaggtgcagctggtggagtctggcggcggactggtgcagcccggcggcagcctgcgcctgtcctgcgctgcctccggctacaccttcaccaactacggcatgaactgggtgaggcaggcccccggaaagggcctggagtgggtgggctggatcaacacctacaccggcgagcccacctacgccgctgactttaagcgcaggtttaccttctccctggacacctccaagtccaccgcctacctgcagatgaacagcctgagggccgaggacaccgccgtgtactactgcgccaagtacccccactactatggctccagccactggtactttgacgtgtggggccagggcaccctggtcacagtgtctagtgcctccaccaagggcccatcggtcttccccctggcaccctgctccaggagcacctctgagtccacagcggccctgggctgcctggtcaaggactacttccccgaaccggtgacggtgtcgtggaactcaggcgccctgaccagcggcgtgcacaccttcccggctgtcctacagtcctcaggactctactccctcagcagcgtggtgaccgtgccctccagcagcttgggcaccaagacatatacctgtaatgtggatcacaagccttccaatacaaaagtggacaagagagttgagtccaagtacggcccaccatgtcctccatgtccagcccctgaatttttgggcgggccttctgtctttctgtttcctcctaaacctaaagataccctgatgatcagccgcacacccgaagtcacttgtgtggtcgtggatgtgtctcaggaagatcccgaagtgcagtttaactggtatgtcgatggcgtggaagtgcataatgccaaaactaagccccgcgaagaacagttcaacagcacttatcgggtcgtgtctgtgctcacagtcctccatcaggattggctgaatgggaaagaatataagtgcaaggtgagcaataagggcctccccagcagcatcgagaagactattagcaaagccaaagggcagccacgggaaccccaggtgtacactctgcccccctctcaggaggagatgactaaaaatcaggtctctctgacttgtctggtgaaagggttttatcccagcgacattgccgtggagtgggagtctaatggccagcccgagaataattataagacaactccccccgtcctggactctgacggcagctttttcctgtattctcggctgacagtggacaaaagtcgctggcaggagggcaatgtctttagttgcagtgtcatgcatgaggccctgcacaatcactatacacagaaaagcctgtctctgagtctgggcaaa

SEQ ID NO: 18 - protein, 681 aa, Homo
EVQLVESGGGLVQPGGSLRLSCAASGYTFTNYGMNWVRQAPGKGLEWVGWINTYTGEPTYAADFKRRFTFSLDTSKSTAYLQMNSLRAEDTAVYYCAKYPHYYGSSHWYFDVWGQGTLVTVSSASTKGPSVFPLAPCSRSTSESTAALGCLVKDYFPEPVTVSWNSGALTSGVHTFPAVLQSSGLYSLSSVVTVPSSSLGTKTYTCNVDHKPSNTKVDKRVGGGGSGGGGSGGGGSEVQLVESGGGLVQPGGSLRLSCAASGFVFSNYDMSWVRQAPGKRLEWVATISGGGGYTYYSDSVKGRFTISRDNAKNSLYLQMNSLRAEDTAVYYCASPYGHYGFEYWGQGTLVTVSSASTKGPSVFPLAPCSRSTSESTAALGCLVKDYFPEPVTVSWNSGALTSGVHTFPAVLQSSGLYSLSSVVTVPSSSLGTKTYTCNVDHKPSNTKVDKRVESKYGPPCPPCPAPEFLGGPSVFLFPPKPKDTLMISRTPEVTCVVVDVSQEDPEVQFNWYVDGVEVHNAKTKPREEQFNSTYRVVSVLTVLHQDWLNGKEYKCKVSNKGLPSSIEKTISKAKGQPREPQVYTLPPSQEEMTKNQVSLTCLVKGFYPSDIAVEWESNGQPENNYKTTPPVLDSDGSFFLYSRLTVDKSRWQEGNVFSCSVMHEALHNHYTQKSLSLSLGK

SEQ ID NO: 19 - DNA, 2043 bp, Homo
gaggtgcagctggtggagtctggcggcggactggtgcagcccggcggcagcctgcgcctgtcctgcgctgcctccggctacaccttcaccaactacggcatgaactgggtgaggcaggcccccggaaagggcctggagtgggtgggctggatcaacacctacaccggcgagcccacctacgccgctgactttaagcgcaggtttaccttctccctggacacctccaagtccaccgcctacctgcagatgaacagcctgagggccgaggacaccgccgtgtactactgcgccaagtacccccactactatggctccagccactggtactttgacgtgtggggccagggcaccctggtgactgtgagcagcgcaagtaccaagggacctagtgttttccctcttgcaccttgctccaggtcaacatcagagtccacagctgctcttggatgtctcgttaaggactacttcccagagccagttaccgtatcctggaactccggagctttgacaagcggcgttcatacattcccagctgtgttgcagagttctgggttgtacagtttgagctcagtggtgaccgtgccttcatcttctttgggcactaagacctacacctgcaacgtggatcacaagccaagcaacaccaaggtggataagagggtgggtggaggcggttcaggcggaggtggcagcggaggtggcgggagtgaggtccagctggtggagagcggaggaggactggtgcagcccggcggctctctgaggctgagctgtgccgctagcggcttcgtcttctccaactacgacatgagctgggtgaggcaagcccccggcaagaggctggagtgggtggctacaatcagcggcggcggaggctacacatactactccgactccgtgaagggaaggttcactatctctagggacaacgccaagaactctctgtatctgcagatgaactctctgagagccgaggatacagctgtgtactactgtgcctccccatacggccactacggcttcgagtactggggccaaggcactctggtcacagtgtctagtgcctccaccaagggcccatcggtcttccccctggcaccctgctccaggagcacctctgagtccacagcggccctgggctgcctggtcaaggactacttccccgaaccggtgacggtgtcgtggaactcaggcgccctgaccagcggcgtgcacaccttcccggctgtcctacagtcctcaggactctactccctcagcagcgtggtgaccgtgccctccagcagcttgggcaccaagacatatacctgtaatgtggatcacaagccttccaatacaaaagtggacaagagagttgagtccaagtacggcccaccatgtcctccatgtccagcccctgaatttttgggcgggccttctgtctttctgtttcctcctaaacctaaagataccctgatgatcagccgcacacccgaagtcacttgtgtggtcgtggatgtgtctcaggaagatcccgaagtgcagtttaactggtatgtcgatggcgtggaagtgcataatgccaaaactaagccccgcgaagaacagttcaacagcacttatcgggtcgtgtctgtgctcacagtcctccatcaggattggctgaatgggaaagaatataagtgcaaggtgagcaataagggcctccccagcagcatcgagaagactattagcaaagccaaagggcagccacgggaaccccaggtgtacactctgcccccctctcaggaggagatgactaaaaatcaggtctctctgacttgtctggtgaaagggttttatcccagcgacattgccgtggagtgggagtctaatggccagcccgagaataattataagacaactccccccgtcctggactctgacggcagctttttcctgtattctcggctgacagtggacaaaagtcgctggcaggagggcaatgtctttagttgcagtgtcatgcatgaggccctgcacaatcactatacacagaaaagcctgtctctgagtctgggcaaa

SEQ ID NO: 20 - protein, 123 aa, Homo [sequence omitted]

SEQ ID NO: 21 - protein, 681 aa, Homo
EVQLVESGGGLVQPGGSLRLSCAASGFVFSNYDMSWVRQAPGKRLEWVATISGGGGYTYYSDSVKGRFTISRDNAKNSLYLQMNSLRAEDTAVYYCASPYGHYGFEYWGQGTLVTVSSASTKGPSVFPLAPCSRSTSESTAALGCLVKDYFPEPVTVSWNSGALTSGVHTFPAVLQSSGLYSLSSVVTVPSSSLGTKTYTCNVDHKPSNTKVDKRVGGGGSGGGGSGGGGSEVQLVESGGGLVQPGGSLRLSCAASGYDFTHYGMNWVRQAPGKGLEWVGWINTYTGEPTYAADFKRRFTFSLDTSKSTAYLQMNSLRAEDTAVYYCAKYPYYYGTSHWYFDVWGQGTLVTVSSASTKGPSVFPLAPCSRSTSESTAALGCLVKDYFPEPVTVSWNSGALTSGVHTFPAVLQSSGLYSLSSVVTVPSSSLGTKTYTCNVDHKPSNTKVDKRVESKYGPPCPPCPAPEFLGGPSVFLFPPKPKDTLMISRTPEVTCVVVDVSQEDPEVQFNWYVDGVEVHNAKTKPREEQFNSTYRVVSVLTVLHQDWLNGKEYKCKVSNKGLPSSIEKTISKAKGQPREPQVYTLPPSQEEMTKNQVSLTCLVKGFYPSDIAVEWESNGQPENNYKTTPPVLDSDGSFFLYSRLTVDKSRWQEGNVFSCSVMHEALHNHYTQKSLSLSLGK

SEQ ID NO: 22 - DNA, 2043 bp, Homo
gaggtccagctggtggagagcggaggaggactggtgcagcccggcggctctctgaggctgagctgtgccgctagcggcttcgtcttctccaactacgacatgagctgggtgaggcaagcccccggcaagaggctggagtgggtggctacaatcagcggcggcggaggctacacatactactccgactccgtgaagggaaggttcactatctctagggacaacgccaagaactctctgtatctgcagatgaactctctgagagccgaggatacagctgtgtactactgtgcctccccatacggccactacggcttcgagtactggggccaaggcactctggtcactgtgagcagcgcaagtaccaagggacctagtgttttccctcttgcaccttgctccaggtcaacatcagagtccacagctgctcttggatgtctcgttaaggactacttcccagagccagttaccgtatcctggaactccggagctttgacaagcggcgttcatacattcccagctgtgttgcagagttctgggttgtacagtttgagctcagtggtgaccgtgccttcatcttctttgggcactaagacctacacctgcaacgtggatcacaagccaagcaacaccaaggtggataagagggtgggtggaggcggttcaggcggaggtggcagcggaggtggcgggagtgaggtgcagctggtggagtctggaggaggcctggtgcagcctggcggctctctgagactgtcttgcgctgctagtggatatgattttacacattatggcatgaactgggtgagacaggctccaggcaagggcctggaatgggtgggctggattaatacctatacaggcgaacctacctacgccgctgattttaagagaagattcaccttttctctggatacatctaagagcacagcttacctgcagatgaacagcctgcgggccgaggacaccgccgtgtactactgcgccaagtacccctactactacggcacctcccactggtacttcgacgtgtggggccagggcaccctggtgaccgtgtcctccgcctccaccaagggcccatcggtcttccccctggcaccctgctccaggagcacctctgagtccacagcggccctgggctgcctggtcaaggactacttccccgaaccggtgacggtgtcgtggaactcaggcgccctgaccagcggcgtgcacaccttcccggctgtcctacagtcctcaggactctactccctcagcagcgtggtgaccgtgccctccagcagcttgggcaccaagacatatacctgtaatgtggatcacaagccttccaatacaaaagtggacaagagagttgagtccaagtacggcccaccatgtcctccatgtccagcccctgaatttttgggcgggccttctgtctttctgtttcctcctaaacctaaagataccctgatgatcagccgcacacccgaagtcacttgtgtggtcgtggatgtgtctcaggaagatcccgaagtgcagtttaactggtatgtcgatggcgtggaagtgcataatgccaaaactaagccccgcgaagaacagttcaacagcacttatcgggtcgtgtctgtgctcacagtcctccatcaggattggctgaatgggaaagaatataagtgcaaggtgagcaataagggcctccccagcagcatcgagaagactattagcaaagccaaagggcagccacgggaaccccaggtgtacactctgcccccctctcaggaggagatgactaaaaatcaggtctctctgacttgtctggtgaaagggttttatcccagcgacattgccgtggagtgggagtctaatggccagcccgagaataattataagacaactccccccgtcctggactctgacggcagctttttcctgtattctcggctgacagtggacaaaagtcgctggcaggagggcaatgtctttagttgcagtgtcatgcatgaggccctgcacaatcactatacacagaaaagcctgtctctgagtctgggcaaa

SEQ ID NO: 23 - protein, 5 aa, Mus musculus
TYWMN

SEQ ID NO: 24 - protein, 17 aa, Mus musculus
QIFPASGSTNYNEMFEG

SEQ ID NO: 25 - protein, 12 aa, Mus musculus
GDGNYALDAMDY

SEQ ID NO: 26 - protein, 15 aa, Mus musculus
RASESVDSYGNSFMH

SEQ ID NO: 27 - protein, 7 aa, Mus musculus
LASNLES

SEQ ID NO: 28 - protein, 9 aa, Mus musculus
QQNNEDPLT

SEQ ID NO: 29 - protein, 121 aa, Homo
QVQLVQSGAEVKKPGASVKVSCKASGYIFITYWMNWVRQAPGQGLEWIGQIFPASGSTNYNEMFEGRATLTVDTSTSTAYMELSSLRSEDTAVYYCARGDGNYALDAMDYWGQGTLVTVSS

SEQ ID NO: 30 - protein, 111 aa, Homo
DIVLTQSPASLAVSPGQRATITCRASESVDSYGNSFMHWYQQKPGQPPKLLIYLASNLESGVPARFSGSGSGTDFTLTINPVEADDTANYYCQQNNEDPLTFGGGTKVELK

SEQ ID NO: 31 - protein, 121 aa, Homo
QVQLVQSGAEVKKPGASVKVSCKASGYTFTSEWMNWVRQAPGQGLEWMGQIFPALGSTNYNEMYEGRVTMTTDTSTSTAYMELRSLRSDDTAVYYCARGIGNYALDAMDYWGQGTLVTVSS

SEQ ID NO: 32 - protein, 111 aa, Homo
DIQMTQSPSSLSASVGDRVTITCRASESVDFYGNSFMHWYQQKPGKAPKLLIYLASNLESGVPSRFSGSGSGTDFTLTISSLQPEDFATYYCQQNIEDPLTFGGGTKVEIK

SEQ ID NO: 33 - protein, 116 aa, Mus musculus
EVQLQQSGPELVKPGASMKISCKASGYSFTGYTMNWVKQSHGKTLEWIGLINPYNGDTSYNQKFKGKATVTVDKSSSTAYMELLNLTSEDSAVYYCARWRYTMDYWGQGTSVTVSS

SEQ ID NO: 34 - protein, 111 aa, Mus musculus
NIALTQSPASVAVSLGQRATISCRASESVDNYGNSFMNWYQQKPGQPPKPLIYFASNLESGVPARFSGSGSRTDFTLTIDPVEADDAATYYCQQNNEAPPTFGGGTKLEIK

SEQ ID NO: 35 - protein, 5 aa, Mus musculus
GYTMN

SEQ ID NO: 36 - protein, 17 aa, Mus musculus
LINPYNGDTSYNQKFKG

SEQ ID NO: 37 - protein, 7 aa, Mus musculus
WRYTMDY

SEQ ID NO: 38 - protein, 15 aa, Mus musculus
RASESVDNYGNSFMN

SEQ ID NO: 39 - protein, 7 aa, Mus musculus
FASNLES

SEQ ID NO: 40 - protein, 9 aa, Mus musculus
QQNNEAPPT

SEQ ID NO: 41 - protein, 116 aa, Homo
QVQLVQSGAEVKKPGASVKVSCKASGYSFTGYTMNWVRQAPGQGLEWIGLINPYNGDTSYNQKFKGRATVTVDKSTSTAYMELSSLRSEDTAVYYCARWRYTMDYWGQGTLVTVSS

SEQ ID NO: 42 - protein, 111 aa, Homo
DIVLTQSPASLAVSPGQRATITCRASESVDNYGNSFMNWYQQKPGQPPKPLIYFASNLESGVPARFSGSGSRTDFTLTINPVEADDTANYYCQQNNEAPPTFGQGTKVEIK

SEQ ID NO: 43 - protein, 218 aa, Homo
DIVLTQSPASLAVSPGQRATITCRASESVDNYGNSFMNWYQQKPGQPPKPLIYFASNLESGVPARFSGSGSRTDFTLTINPVEADDTANYYCQQNNEAPPTFGQGTKVEIKRTVAAPSVFIFPPSDEQLKSGTASVVCLLNNFYPREAKVQWKVDNALQSGNSQESVTEQDSKDSTYSLSSTLTLSKADYEKHKVYACEVTHQGLSSPVTKSFNRGEC

SEQ ID NO: 44 - DNA, 654 bp, Homo
gatatcgtgctgactcagagcccagcctctctggctgtgagccccggccagagagccacaatcacttgtagggccagcgagagcgtggacaactacggcaactccttcatgaattggtaccagcagaagcccggccagcctccaaagcctctgatctacttcgcctccaatctggaaagcggcgtgccagctaggtttagcggctccggctctaggacagacttcactctgactatcaacccagtggaggccgatgacacagccaactactactgccagcagaacaacgaggcccctccaactttcggccaaggcactaaggtcgagatcaagagaaccgtcgccgctcccagcgtcttcatcttcccccccagcgatgagcagctgaagagcggaaccgccagcgtggtgtgcctgctgaacaacttctaccccagggaggccaaggtgcaatggaaggtggacaacgccctacagagcggcaactcccaggagagcgtgaccgagcaggacagcaaggatagcacctacagcctgagcagcaccctcaccctgagcaaggccgactacgagaagcacaaggtgtacgcctgcgaggtgacccatcagggcctgagcagccctgtgaccaagagcttcaacaggggcgagtgc

SEQ ID NO: 45 - protein, 677 aa, Homo
QVQLVQSGAEVKKPGASVKVSCKASGYSFTGYTMNWVRQAPGQGLEWIGLINPYNGDTSYNQKFKGRATVTVDKSTSTAYMELSSLRSEDTAVYYCARWRYTMDYWGQGTLVTVSSASTKGPSVFPLAPCSRSTSESTAALGCLVKDYFPEPVTVSWNSGALTSGVHTFPAVLQSSGLYSLSSVVTVPSSSLGTKTYTCNVDHKPSNTKVDKRVGGGGSGGGGSGGGGSQVQLVQSGAEVKKPGASVKVSCKASGYIFITYWMNWVRQAPGQGLEWIGQIFPASGSTNYNEMFEGRATLTVDTSTSTAYMELSSLRSEDTAVYYCARGDGNYALDAMDYWGQGTLVTVSSASTKGPSVFPLAPCSRSTSESTAALGCLVKDYFPEPVTVSWNSGALTSGVHTFPAVLQSSGLYSLSSVVTVPSSSLGTKTYTCNVDHKPSNTKVDKRVESKYGPPCPPCPAPEFLGGPSVFLFPPKPKDTLMISRTPEVTCVVVDVSQEDPEVQFNWYVDGVEVHNAKTKPREEQFNSTYRVVSVLTVLHQDWLNGKEYKCKVSNKGLPSSIEKTISKAKGQPREPQVYTLPPSQEEMTKNQVSLTCLVKGFYPSDIAVEWESNGQPENNYKTTPPVLDSDGSFFLYSRLTVDKSRWQEGNVFSCSVMHEALHNHYTQKSLSLSLGK

SEQ ID NO: 46 - DNA, 2031 bp, Homo
caagtgcagctggtccagagcggcgctgaggtgaagaagcccggcgccagcgtgaaagtcagctgcaaagctagcggctactccttcactggctacactatgaactgggtgaggcaagcccccggccaaggcctcgagtggatcggactgatcaacccatacaacggcgacacaagctacaaccagaagttcaagggaagggccacagtgactgtggacaagtccacaagcactgcctacatggaactgagctctctgaggagcgaggatacagccgtgtactactgcgctaggtggagatacacaatggactattggggccaaggcactctggtcactgtgagcagcgcaagtaccaagggacctagtgttttccctcttgcaccttgctccaggtcaacatcagagtccacagctgctcttggatgtctcgttaaggactacttcccagagccagttaccgtatcctggaactccggagctttgacaagcggcgttcatacattcccagctgtgttgcagagttctgggttgtacagtttgagctcagtggtgaccgtgccttcatcttctttgggcactaagacctacacctgcaacgtggatcacaagccaagcaacaccaaggtggataagagggtgggtggaggcggttcaggcggaggtggcagcggaggtggcgggagtcaggtgcagctggtgcagtctggagctgaggtgaagaagcctggcgcttctgtgaaggtgtcttgtaaggcttctggatatatctttattacctattggatgaattgggtgagacaggctcctggccagggcctggagtggatcggacagatttttccagcttctggctccacaaattataatgagatgtttgagggcagagctacactgacagtggatacatctacatctaccgcctacatggaactgtcttctctgagatctgaggatacagctgtgtactattgtgctagaggcgatggcaattatgctctggatgctatggattattggggccagggaacactggtgaccgtgtcttctgcctccaccaagggcccatcggtcttccccctggcaccctgctccaggagcacctctgagtccacagcggccctgggctgcctggtcaaggactacttccccgaaccggtgacggtgtcgtggaactcaggcgccctgaccagcggcgtgcacaccttcccggctgtcctacagtcctcaggactctactccctcagcagcgtggtgaccgtgccctccagcagcttgggcaccaagacatatacctgtaatgtggatcacaagccttccaatacaaaagtggacaagagagttgagtccaagtacggcccaccatgtcctccatgtccagcccctgaatttttgggcgggccttctgtctttctgtttcctcctaaacctaaagataccctgatgatcagccgcacacccgaagtcacttgtgtggtcgtggatgtgtctcaggaagatcccgaagtgcagtttaactggtatgtcgatggcgtggaagtgcataatgccaaaactaagccccgcgaagaacagttcaacagcacttatcgggtcgtgtctgtgctcacagtcctccatcaggattggctgaatgggaaagaatataagtgcaaggtgagcaataagggcctccccagcagcatcgagaagactattagcaaagccaaagggcagccacgggaaccccaggtgtacactctgcccccctctcaggaggagatgactaaaaatcaggtctctctgacttgtctggtgaaagggttttatcccagcgacattgccgtggagtgggagtctaatggccagcccgagaataattataagacaactccccccgtcctggactctgacggcagctttttcctgtattctcggctgacagtggacaaaagtcgctggcaggagggcaatgtctttagttgcagtgtcatgcatgaggccctgcacaatcactatacacagaaaagcctgtctctgagtctgggcaaa

SEQ ID NO: 47 - protein, 677 aa, Homo
QVQLVQSGAEVKKPGASVKVSCKASGYIFITYWMNWVRQAPGQGLEWIGQIFPASGSTNYNEMFEGRATLTVDTSTSTAYMELSSLRSEDTAVYYCARGDGNYALDAMDYWGQGTLVTVSSASTKGPSVFPLAPCSRSTSESTAALGCLVKDYFPEPVTVSWNSGALTSGVHTFPAVLQSSGLYSLSSVVTVPSSSLGTKTYTCNVDHKPSNTKVDKRVGGGGSGGGGSGGGGSQVQLVQSGAEVKKPGASVKVSCKASGYSFTGYTMNWVRQAPGQGLEWIGLINPYNGDTSYNQKFKGRATVTVDKSTSTAYMELSSLRSEDTAVYYCARWRYTMDYWGQGTLVTVSSASTKGPSVFPLAPCSRSTSESTAALGCLVKDYFPEPVTVSWNSGALTSGVHTFPAVLQSSGLYSLSSVVTVPSSSLGTKTYTCNVDHKPSNTKVDKRVESKYGPPCPPCPAPEFLGGPSVFLFPPKPKDTLMISRTPEVTCVVVDVSQEDPEVQFNWYVDGVEVHNAKTKPREEQFNSTYRVVSVLTVLHQDWLNGKEYKCKVSNKGLPSSIEKTISKAKGQPREPQVYTLPPSQEEMTKNQVSLTCLVKGFYPSDIAVEWESNGQPENNYKTTPPVLDSDGSFFLYSRLTVDKSRWQEGNVFSCSVMHEALHNHYTQKSLSLSLGK

SEQ ID NO: 48 - DNA, 2031 bp, Homo
caggtgcagctggtgcagtctggagctgaggtgaagaagcctggcgcttctgtgaaggtgtcttgtaaggcttctggatatatctttattacctattggatgaattgggtgagacaggctcctggccagggcctggagtggatcggacagatttttccagcttctggctccacaaattataatgagatgtttgagggcagagctacactgacagtggatacatctacatctaccgcctatatggagctgtcttctctgagatctgaagataccgctgtgtattattgtgctagaggagatggcaactatgctctggatgccatggattactggggccagggcaccctggtgactgtgagcagcgcaagtaccaagggacctagtgttttccctcttgcaccttgctccaggtcaacatcagagtccacagctgctcttggatgtctcgttaaggactacttcccagagccagttaccgtatcctggaactccggagctttgacaagcggcgttcatacattcccagctgtgttgcagagttctgggttgtacagtttgagctcagtggtgaccgtgccttcatcttctttgggcactaagacctacacctgcaacgtggatcacaagccaagcaacaccaaggtggataagagggtgggtggaggcggttcaggcggaggtggcagcggaggtggcgggagtcaagtgcagctggtccagagcggcgctgaggtgaagaagcccggcgccagcgtgaaagtcagctgcaaagctagcggctactccttcactggctacactatgaactgggtgaggcaagcccccggccaaggcctcgagtggatcggactgatcaacccatacaacggcgacacaagctacaaccagaagttcaagggaagggccacagtgactgtggacaagtccacaagcactgcctacatggaactgagctctctgaggagcgaggatacagccgtgtactactgcgctaggtggagatacacaatggactattggggccaaggcactctggtcacagtgtctagtgcctccaccaagggcccatcggtcttccccctggcaccctgctccaggagcacctctgagtccacagcggccctgggctgcctggtcaaggactacttccccgaaccggtgacggtgtcgtggaactcaggcgccctgaccagcggcgtgcacaccttcccggctgtcctacagtcctcaggactctactccctcagcagcgtggtgaccgtgccctccagcagcttgggcaccaagacatatacctgtaatgtggatcacaagccttccaatacaaaagtggacaagagagttgagtccaagtacggcccaccatgtcctccatgtccagcccctgaatttttgggcgggccttctgtctttctgtttcctcctaaacctaaagataccctgatgatcagccgcacacccgaagtcacttgtgtggtcgtggatgtgtctcaggaagatcccgaagtgcagtttaactggtatgtcgatggcgtggaagtgcataatgccaaaactaagccccgcgaagaacagttcaacagcacttatcgggtcgtgtctgtgctcacagtcctccatcaggattggctgaatgggaaagaatataagtgcaaggtgagcaataagggcctccccagcagcatcgagaagactattagcaaagccaaagggcagccacgggaaccccaggtgtacactctgcccccctctcaggaggagatgactaaaaatcaggtctctctgacttgtctggtgaaagggttttatcccagcgacattgccgtggagtgggagtctaatggccagcccgagaataattataagacaactccccccgtcctggactctgacggcagctttttcctgtattctcggctgacagtggacaaaagtcgctggcaggagggcaatgtctttagttgcagtgtcatgcatgaggccctgcacaatcactatacacagaaaagcctgtctctgagtctgggcaaa

SEQ ID NO: 49 - protein, 677 aa, Homo
QVQLVQSGAEVKKPGASVKVSCKASGYSFTGYTMNWVRQAPGQGLEWIGLINPYNGDTSYNQKFKGRATVTVDKSTSTAYMELSSLRSEDTAVYYCARWRYTMDYWGQGTLVTVSSASTKGPSVFPLAPCSRSTSESTAALGCLVKDYFPEPVTVSWNSGALTSGVHTFPAVLQSSGLYSLSSVVTVPSSSLGTKTYTCNVDHKPSNTKVDKRVGGGGSGGGGSGGGGSQVQLVQSGAEVKKPGASVKVSCKASGYTFTSEWMNWVRQAPGQGLEWMGQIFPALGSTNYNEMYEGRVTMTTDTSTSTAYMELRSLRSDDTAVYYCARGIGNYALDAMDYWGQGTLVTVSSASTKGPSVFPLAPCSRSTSESTAALGCLVKDYFPEPVTVSWNSGALTSGVHTFPAVLQSSGLYSLSSVVTVPSSSLGTKTYTCNVDHKPSNTKVDKRVESKYGPPCPPCPAPEFLGGPSVFLFPPKPKDTLMISRTPEVTCVVVDVSQEDPEVQFNWYVDGVEVHNAKTKPREEQFNSTYRVVSVLTVLHQDWLNGKEYKCKVSNKGLPSSIEKTISKAKGQPREPQVYTLPPSQEEMTKNQVSLTCLVKGFYPSDIAVEWESNGQPENNYKTTPPVLDSDGSFFLYSRLTVDKSRWQEGNVFSCSVMHEALHNHYTQKSLSLSLGK

SEQ ID NO: 50 - DNA, 2031 bp, Homo
caagtgcagctggtccagagcggcgctgaggtgaagaagcccggcgccagcgtgaaagtcagctgcaaagctagcggctactccttcactggctacactatgaactgggtgaggcaagcccccggccaaggcctcgagtggatcggactgatcaacccatacaacggcgacacaagctacaaccagaagttcaagggaagggccacagtgactgtggacaagtccacaagcactgcctacatggaactgagctctctgaggagcgaggatacagccgtgtactactgcgctaggtggagatacacaatggactattggggccaaggcactctggtcactgtgagcagcgcaagtaccaagggacctagtgttttccctcttgcaccttgctccaggtcaacatcagagtccacagctgctcttggatgtctcgttaaggactacttcccagagccagttaccgtatcctggaactccggagctttgacaagcggcgttcatacattcccagctgtgttgcagagttctgggttgtacagtttgagctcagtggtgaccgtgccttcatcttctttgggcactaagacctacacctgcaacgtggatcacaagccaagcaacaccaaggtggataagagggtgggtggaggcggttcaggcggaggtggcagcggaggtggcgggagtcaagtgcagctggtgcagagcggcgctgaggtcaaaaagcccggcgcctccgtgaaggtgagctgtaaggccagcggctacacattcactagcgagtggatgaactgggtgagacaagcccccggccaaggactggaatggatgggccagatcttcccagctctgggctccactaactacaacgagatgtacgagggaagggtcactatgactacagacactagcactagcactgcctacatggaactgaggtctctgagaagcgacgatacagccgtgtactactgcgccagaggcatcggcaactatgctctggatgccatggactactggggccaaggcactctcgtgactgtgagctccgcctccaccaagggcccatcggtcttccccctggcaccctgctccaggagcacctctgagtccacagcggccctgggctgcctggtcaaggactacttccccgaaccggtgacggtgtcgtggaactcaggcgccctgaccagcggcgtgcacaccttcccggctgtcctacagtcctcaggactctactccctcagcagcgtggtgaccgtgccctccagcagcttgggcaccaagacatatacctgtaatgtggatcacaagccttccaatacaaaagtggacaagagagttgagtccaagtacggcccaccatgtcctccatgtccagcccctgaatttttgggcgggccttctgtctttctgtttcctcctaaacctaaagataccctgatgatcagccgcacacccgaagtcacttgtgtggtcgtggatgtgtctcaggaagatcccgaagtgcagtttaactggtatgtcgatggcgtggaagtgcataatgccaaaactaagccccgcgaagaacagttcaacagcacttatcgggtcgtgtctgtgctcacagtcctccatcaggattggctgaatgggaaagaatataagtgcaaggtgagcaataagggcctccccagcagcatcgagaagactattagcaaagccaaagggcagccacgggaaccccaggtgtacactctgcccccctctcaggaggagatgactaaaaatcaggtctctctgacttgtctggtgaaagggttttatcccagcgacattgccgtggagtgggagtctaatggccagcccgagaataattataagacaactccccccgtcctggactctgacggcagctttttcctgtattctcggctgacagtggacaaaagtcgctggcaggagggcaatgtctttagttgcagtgtcatgcatgaggccctgcacaatcactatacacagaaaagcctgtctctgagtctgggcaaa

SEQ ID NO: 51 - protein, 677 aa, Homo
QVQLVQSGAEVKKPGASVKVSCKASGYTFTSEWMNWVRQAPGQGLEWMGQIFPALGSTNYNEMYEGRVTMTTDTSTSTAYMELRSLRSDDTAVYYCARGIGNYALDAMDYWGQGTLVTVSSASTKGPSVFPLAPCSRSTSESTAALGCLVKDYFPEPVTVSWNSGALTSGVHTFPAVLQSSGLYSLSSVVTVPSSSLGTKTYTCNVDHKPSNTKVDKRVGGGGSGGGGSGGGGSQVQLVQSGAEVKKPGASVKVSCKASGYSFTGYTMNWVRQAPGQGLEWIGLINPYNGDTSYNQKFKGRATVTVDKSTSTAYMELSSLRSEDTAVYYCARWRYTMDYWGQGTLVTVSSASTKGPSVFPLAPCSRSTSESTAALGCLVKDYFPEPVTVSWNSGALTSGVHTFPAVLQSSGLYSLSSVVTVPSSSLGTKTYTCNVDHKPSNTKVDKRVESKYGPPCPPCPAPEFLGGPSVFLFPPKPKDTLMISRTPEVTCVVVDVSQEDPEVQFNWYVDGVEVHNAKTKPREEQFNSTYRVVSVLTVLHQDWLNGKEYKCKVSNKGLPSSIEKTISKAKGQPREPQVYTLPPSQEEMTKNQVSLTCLVKGFYPSDIAVEWESNGQPENNYKTTPPVLDSDGSFFLYSRLTVDKSRWQEGNVFSCSVMHEALHNHYTQKSLSLSLGK

SEQ ID NO: 52 - DNA, 2031 bp, Homo
caagtgcagctggtgcagagcggcgctgaggtcaaaaagcccggcgcctccgtgaaggtgagctgtaaggccagcggctacacattcactagcgagtggatgaactgggtgagacaagcccccggccaaggactggaatggatgggccagatcttcccagctctgggctccactaactacaacgagatgtacgagggaagggtcactatgactacagacactagcactagcactgcctacatggaactgaggtctctgagaagcgacgatacagccgtgtactactgcgccagaggcatcggcaactatgctctggatgccatggactactggggccaaggcactctcgtgactgtgagctccgcaagtaccaagggacctagtgttttccctcttgcaccttgctccaggtcaacatcagagtccacagctgctcttggatgtctcgttaaggactacttcccagagccagttaccgtatcctggaactccggagctttgacaagcggcgttcatacattcccagctgtgttgcagagttctgggttgtacagtttgagctcagtggtgaccgtgccttcatcttctttgggcactaagacctacacctgcaacgtggatcacaagccaagcaacaccaaggtggataagagggtgggtggaggcggttcaggcggaggtggcagcggaggtggcgggagtcaagtgcagctggtccagagcggcgctgaggtgaagaagcccggcgccagcgtgaaagtcagctgcaaagctagcggctactccttcactggctacactatgaactgggtgaggcaagcccccggccaaggcctcgagtggatcggactgatcaacccatacaacggcgacacaagctacaaccagaagttcaagggaagggccacagtgactgtggacaagtccacaagcactgcctacatggaactgagctctctgaggagcgaggatacagccgtgtactactgcgctaggtggagatacacaatggactattggggccaaggcactctggtcacagtgtctagtgcctccaccaagggcccatcggtcttccccctggcaccctgctccaggagcacctctgagtccacagcggccctgggctgcctggtcaaggactacttccccgaaccggtgacggtgtcgtggaactcaggcgccctgaccagcggcgtgcacaccttcccggctgtcctacagtcctcaggactctactccctcagcagcgtggtgaccgtgccctccagcagcttgggcaccaagacatatacctgtaatgtggatcacaagccttccaatacaaaagtggacaagagagttgagtccaagtacggcccaccatgtcctccatgtccagcccctgaatttttgggcgggccttctgtctttctgtttcctcctaaacctaaagataccctgatgatcagccgcacacccgaagtcacttgtgtggtcgtggatgtgtctcaggaagatcccgaagtgcagtttaactggtatgtcgatggcgtggaagtgcataatgccaaaactaagccccgcgaagaacagttcaacagcacttatcgggtcgtgtctgtgctcacagtcctccatcaggattggctgaatgggaaagaatataagtgcaaggtgagcaataagggcctccccagcagcatcgagaagactattagcaaagccaaagggcagccacgggaaccccaggtgtacactctgcccccctctcaggaggagatgactaaaaatcaggtctctctgacttgtctggtgaaagggttttatcccagcgacattgccgtggagtgggagtctaatggccagcccgagaataattataagacaactccccccgtcctggactctgacggcagctttttcctgtattctcggctgacagtggacaaaagtcgctggcaggagggcaatgtctttagttgcagtgtcatgcatgaggccctgcacaatcactatacacagaaaagcctgtctctgagtctgggcaaa

SEQ ID NO: 53 - protein, 117 aa, Homo
QVQLVQSGAEVKKPGASVKVSCKGSGYTFTDYAIHWVRQAPGQSLEWIGVFSIYYENINYNQKFKGRATMTVDKSTSTAYMELRSLRSDDTAVYYCARRDGGTINYWGQGTLVTVSS

SEQ ID NO: 54 - protein, 112 aa, Homo
DVVMTQSPLSLPVTLGQPASISCRSSQSLVHSNGNTYLHWYQQRPGQSPRLLIYKVSNRFSGVPDRFSGSGSGTDFTLKISRVEAEDVGVYFCSQSTHIPWTFGQGTKVEIK

SEQ ID NO: 55 - protein, 5 aa, Mus musculus
NHVIH

SEQ ID NO: 56 - protein, 17 aa, Mus musculus
YIYPYNDGTKYNEKFKD

SEQ ID NO: 57 - protein, 8 aa, Mus musculus
GGYYTYDD

SEQ ID NO: 58 - protein, 16 aa, Mus musculus
RSSQSLVHSNGKTYLH

SEQ ID NO: 59 - protein, 7 aa, Mus musculus
KVSNRFS

SEQ ID NO: 60 - protein, 9 aa, Mus musculus
SQSTHVPYT

SEQ ID NO: 61 - protein, 117 aa, Homo
QVQLVQSGAEVKKPGASVKVSCKASGYTFANHVIHWVRQAPGQGLEWMGYIYPYNDGTKYNEKFKDRVTLTSDKSTSTVYMELSSLRSEDTAVYYCARGGYYTYDDWGQGTLVTVSS

SEQ ID NO: 62 - protein, 112 aa, Homo
DVVMTQSPLSLPVTLGQPASISCRSSQSLVHSNGKTYLHWYQQRPGQSPRLLIYKVSNRFSGVPDRFSGSGSGTDFTLKISRVEAEDVGVYYCSQSTHVPYTFGQGTKVEIK

SEQ ID NO: 63 - protein, 219 aa, Homo
DVVMTQSPLSLPVTLGQPASISCRSSQSLVHSNGNTYLHWYQQRPGQSPRLLIYKVSNRFSGVPDRFSGSGSGTDFTLKISRVEAEDVGVYFCSQSTHIPWTFGQGTKVEIKRTVAAPSVFIFPPSDEQLKSGTASVVCLLNNFYPREAKVQWKVDNALQSGNSQESVTEQDSKDSTYSLSSTLTLSKADYEKHKVYACEVTHQGLSSPVTKSFNRGEC

SEQ ID NO: 64 - DNA, 657 bp, Homo
gacgtggtgatgacccagagccctttatctttacccgttacactgggacagcccgccagcatcagctgtcgtagcagccagtctttagtgcacagcaacggcaacacctatttacactggtaccagcagagacccggccagagccccagactgctgatctacaaggtgagcaatcgtttctccggcgtgcccgacagattcagcggcagcggaagcggcaccgacttcactttaaagatcagcagagtggaggccgaggacgtgggcgtgtacttctgcagccagagcacccacatcccttggaccttcggccaaggtaccaaggtggagatcaagagaaccgtcgccgctcccagcgtcttcatcttcccccccagcgatgagcagctgaagagcggaaccgccagcgtggtgtgcctgctgaacaacttctaccccagggaggccaaggtgcaatggaaggtggacaacgccctacagagcggcaactcccaggagagcgtgaccgagcaggacagcaaggatagcacctacagcctgagcagcaccctcaccctgagcaaggccgactacgagaagcacaaggtgtacgcctgcgaggtgacccatcagggcctgagcagccctgtgaccaagagcttcaacaggggcgagtgc

SEQ ID NO: 65 - protein, 677 aa, Homo
QVQLVQSGAEVKKPGASVKVSCKASGYTFANHVIHWVRQAPGQGLEWMGYIYPYNDGTKYNEKFKDRVTLTSDKSTSTVYMELSSLRSEDTAVYYCARGGYYTYDDWGQGTLVTVSSASTKGPSVFPLAPCSRSTSESTAALGCLVKDYFPEPVTVSWNSGALTSGVHTFPAVLQSSGLYSLSSVVTVPSSSLGTKTYTCNVDHKPSNTKVDKRVGGGGSGGGGSGGGGSQVQLVQSGAEVKKPGASVKVSCKGSGYTFTDYAIHWVRQAPGQSLEWIGVFSIYYENINYNQKFKGRATMTVDKSTSTAYMELRSLRSDDTAVYYCARRDGGTINYWGQGTLVTVSSASTKGPSVFPLAPSSKSTSGGTAALGCLVKDYFPEPVTVSWNSGALTSGVHTFPAVLQSSGLYSLSSVVTVPSSSLGTQTYICNVNHKPSNTKVDKKVEPKSCDKTHTCPPCPAPELLGGPSVFLFPPKPKDTLMISRTPEVTCVVVDVSHEDPEVKFNWYVDGVEVHNAKTKPREEQYNSTYRVVSVLTVLHQDWLNGKEYKCKVSNKALPAPIEKTISKAKGQPREPQVYTLPPSREEMTKNQVSLTCLVKGFYPSDIAVEWESNGQPENNYKTTPPVLDSDGSFFLYSKLTVDKSRWQQGNVFSCSVMHEALHNHYTQKSLSLSPGK

SEQ ID NO: 66 - DNA, 2031 bp, Homo
caggtgcagctggtgcagtccggcgccgaggtgaagaagcccggcgcctccgtgaaagtgagctgcaaggcatccggctacaccttcgccaaccacgtgatccactgggtgcggcaggcccccggccagggcctggagtggatgggctacatctatccttataatgatggcacaaagtataatgagaagtttaaggatagggtaacactgacatctgataagtctacatctacagtgtacatggagctgtcctctctgaggtccgaggacaccgccgtgtactactgcgccagaggcggctactacacctacgacgactggggccagggcaccctggtgaccgtgtcctccgcaagtaccaagggacctagtgttttccctcttgcaccttgctccaggtcaacatcagagtccacagctgctcttggatgtctcgttaaggactacttcccagagccagttaccgtatcctggaactccggagctttgacaagcggcgttcatacattcccagctgtgttgcagagttctgggttgtacagtttgagctcagtggtgaccgtgccttcatcttctttgggcactaagacctacacctgcaacgtggatcacaagccaagcaacaccaaggtggataagagggtgggtggaggcggttcaggcggaggtggcagcggaggtggcgggagtcaagttcagctggtgcagagcggagctgaggtgaagaagcccggcgccagcgtgaaggtgagctgtaagggcagcggctacaccttcaccgactacgccatccactgggtgagacaagctcccggtcagtctttagaatggatcggcgtgttcagcatctactacgagaacatcaactataaccagaagttcaagggtcgtgccaccatgaccgtggacaagagcaccagcaccgcctacatggagctgaggtctttaaggagcgacgacaccgccgtgtactactgcgctcgtagggacggcggcaccatcaactactggggccaaggtactttagtgacagtgagcagcgcgagcaccaagggaccttccgtgtttcccctcgcccccagctccaaaagcaccagcggcggaacagctgctctcggctgtctcgtcaaggattacttccccgagcccgtgaccgtgagctggaacagcggagccctgacaagcggcgtccacaccttccctgctgtcctacagtcctccggactgtacagcctgagcagcgtggtgacagtccctagcagctccctgggcacccagacatatatttgcaacgtgaatcacaagcccagcaacaccaaggtcgataagaaggtggagcctaagtcctgcgacaagacccacacatgtcccccctgtcccgctcctgaactgctgggaggcccttccgtgttcctgttcccccctaagcccaaggacaccctgatgatttccaggacacccgaggtgacctgtgtggtggtggacgtcagccacgaggaccccgaggtgaaattcaactggtacgtcgatggcgtggaggtgcacaacgctaagaccaagcccagggaggagcagtacaattccacctacagggtggtgtccgtgctgaccgtcctccatcaggactggctgaacggcaaagagtataagtgcaaggtgagcaacaaggccctccctgctcccatcgagaagaccatcagcaaagccaagggccagcccagggaacctcaagtctataccctgcctcccagcagggaggagatgaccaagaaccaagtgagcctcacatgcctcgtcaagggcttctatccttccgatattgccgtcgagtgggagtccaacggacagcccgagaacaactacaagacaacaccccccgtgctcgattccgatggcagcttcttcctgtactccaagctgaccgtggacaagtccagatggcaacaaggcaacgtcttcagttgcagcgtcatgcatgaggccctccacaaccactacacccagaaaagcctgtctctgagtcctggcaaa

SEQ ID NO: 67 - protein, 677 aa, Homo
QVQLVQSGAEVKKPGASVKVSCKGSGYTFTDYAIHWVRQAPGQSLEWIGVFSIYYENINYNQKFKGRATMTVDKSTSTAYMELRSLRSDDTAVYYCARRDGGTINYWGQGTLVTVSSASTKGPSVFPLAPCSRSTSESTAALGCLVKDYFPEPVTVSWNSGALTSGVHTFPAVLQSSGLYSLSSVVTVPSSSLGTKTYTCNVDHKPSNTKVDKRVGGGGSGGGGSGGGGSQVQLVQSGAEVKKPGASVKVSCKASGYTFANHVIHWVRQAPGQGLEWMGYIYPYNDGTKYNEKFKDRVTLTSDKSTSTVYMELSSLRSEDTAVYYCARGGYYTYDDWGQGTLVTVSSASTKGPSVFPLAPSSKSTSGGTAALGCLVKDYFPEPVTVSWNSGALTSGVHTFPAVLQSSGLYSLSSVVTVPSSSLGTQTYICNVNHKPSNTKVDKKVEPKSCDKTHTCPPCPAPELLGGPSVFLFPPKPKDTLMISRTPEVTCVVVDVSHEDPEVKFNWYVDGVEVHNAKTKPREEQYNSTYRVVSVLTVLHQDWLNGKEYKCKVSNKALPAPIEKTISKAKGQPREPQVYTLPPSREEMTKNQVSLTCLVKGFYPSDIAVEWESNGQPENNYKTTPPVLDSDGSFFLYSKLTVDKSRWQQGNVFSCSVMHEALHNHYTQKSLSLSPGK

SEQ ID NO: 68 - DNA, 2031 bp, Homo
caagttcagctggtgcagagcggagctgaggtgaagaagcccggcgccagcgtgaaggtgagctgtaagggcagcggctacaccttcaccgactacgccatccactgggtgagacaagctcccggtcagtctttagaatggatcggcgtgttcagcatctactacgagaacatcaactataaccagaagttcaagggtcgtgccaccatgaccgtggacaagagcaccagcaccgcctacatggagctgaggtctttaaggagcgacgacaccgccgtgtactactgcgctcgtagggacggcggcaccatcaactactggggccaaggtactttagtgacagtgagcagcgcaagtaccaagggacctagtgttttccctcttgcaccttgctccaggtcaacatcagagtccacagctgctcttggatgtctcgttaaggactacttcccagagccagttaccgtatcctggaactccggagctttgacaagcggcgttcatacattcccagctgtgttgcagagttctgggttgtacagtttgagctcagtggtgaccgtgccttcatcttctttgggcactaagacctacacctgcaacgtggatcacaagccaagcaacaccaaggtggataagagggtgggtggaggcggttcaggcggaggtggcagcggaggtggcgggagtcaggtgcagctggtgcagtccggcgccgaggtgaagaagcccggcgcctccgtgaaagtgagctgcaaggcatccggctacaccttcgccaaccacgtgatccactgggtgcggcaggcccccggccagggcctggagtggatgggctacatctatccttataatgatggcacaaagtataatgagaagtttaaggatagggtaacactgacatctgataagtctacatctacagtgtacatggagctgtcctctctgaggtccgaggacaccgccgtgtactactgcgccagaggcggctactacacctacgacgactggggccagggcaccctggtgaccgtgtcctccgcgagcaccaagggaccttccgtgtttcccctcgcccccagctccaaaagcaccagcggcggaacagctgctctcggctgtctcgtcaaggattacttccccgagcccgtgaccgtgagctggaacagcggagccctgacaagcggcgtccacaccttccctgctgtcctacagtcctccggactgtacagcctgagcagcgtggtgacagtccctagcagctccctgggcacccagacatatatttgcaacgtgaatcacaagcccagcaacaccaaggtcgataagaaggtggagcctaagtcctgcgacaagacccacacatgtcccccctgtcccgctcctgaactgctgggaggcccttccgtgttcctgttcccccctaagcccaaggacaccctgatgatttccaggacacccgaggtgacctgtgtggtggtggacgtcagccacgaggaccccgaggtgaaattcaactggtacgtcgatggcgtggaggtgcacaacgctaagaccaagcccagggaggagcagtacaattccacctacagggtggtgtccgtgctgaccgtcctccatcaggactggctgaacggcaaagagtataagtgcaaggtgagcaacaaggccctccctgctcccatcgagaagaccatcagcaaagccaagggccagcccagggaacctcaagtctataccctgcctcccagcagggaggagatgaccaagaaccaagtgagcctcacatgcctcgtcaagggcttctatccttccgatattgccgtcgagtgggagtccaacggacagcccgagaacaactacaagacaacaccccccgtgctcgattccgatggcagcttcttcctgtactccaagctgaccgtggacaagtccagatggcaacaaggcaacgtcttcagttgcagcgtcatgcatgaggccctccacaaccactacacccagaaaagcctgtctctgagtcctggcaaa

SEQ ID NO: 69 - protein, 111 aa, Mus musculus
QVQLKESGPGLVAPSQSLSITCTVSGFSLSSYDISWIRQPPGKGLEWLGVIWTGGGTNYNSAFMSRLSISKDNSKSQVFLKMNSLQTDDTAKYYCVRMDYWGQGTSVTVSS

SEQ ID NO: 70 - protein, 112 aa, Mus musculus
DVVMTQTPLSLPVSLGDQASISCRSSQSLLHSNGNTYLHWYLQKPGQSPKLLFYKVSNRFSGVPDRFSGSGSGTDFTLKISRVEAEDLGVYFCSQSTHVPWTFGGGTKLEIK

SEQ ID NO: 71 - protein, 5 aa, Mus musculus
SYDIS

SEQ ID NO: 72 - protein, 16 aa, Mus musculus
VIWTGGGTNYNSAFMS

SEQ ID NO: 73 - protein, 3 aa, Mus musculus
MDY

SEQ ID NO: 74 - protein, 16 aa, Mus musculus
RSSQSLLHSNGNTYLH

SEQ ID NO: 75 - protein, 7 aa, Mus musculus
KVSNRFS

SEQ ID NO: 76 - protein, 9 aa, Mus musculus
SQSTHVPWT

SEQ ID NO: 77 - protein, 111 aa, Homo
QVQLQESGPGLVKPSETLSLTCTVSGFSLSSYDISWIRQPPGKGLEWLGVIWTGGGTNYNSAFMSRLTISKDNSKSQVSLKLSSVTAADTAVYYCVRMDYWGQGTLVTVSS

SEQ ID NO: 78 - protein, 112 aa, Homo
DVVMTQSPLSLPVTLGQPASISCRSSQSLLHSNGNTYLHWYQQRPGQSPRLLFYKVSNRFSGVPDRFSGSGSGTDFTLKISRVEAEDVGVYFCSQSTHVPWTFGQGTKVEIK

SEQ ID NO: 79 - protein, 671 aa, Homo
QVQLQESGPGLVKPSETLSLTCTVSGFSLSSYDISWIRQPPGKGLEWLGVIWTGGGTNYNSAFMSRLTISKDNSKSQVSLKLSSVTAADTAVYYCVRMDYWGQGTLVTVSSASTKGPSVFPLAPCSRSTSESTAALGCLVKDYFPEPVTVSWNSGALTSGVHTFPAVLQSSGLYSLSSVVTVPSSSLGTKTYTCNVDHKPSNTKVDKRVGGGGSGGGGSGGGGSQVQLVQSGAEVKKPGASVKVSCKGSGYTFTDYAIHWVRQAPGQSLEWIGVFSIYYENINYNQKFKGRATMTVDKSTSTAYMELRSLRSDDTAVYYCARRDGGTINYWGQGTLVTVSSASTKGPSVFPLAPSSKSTSGGTAALGCLVKDYFPEPVTVSWNSGALTSGVHTFPAVLQSSGLYSLSSVVTVPSSSLGTQTYICNVNHKPSNTKVDKKVEPKSCDKTHTCPPCPAPEAAGGPSVFLFPPKPKDTLMISRTPEVTCVVVDVSHEDPEVKFNWYVDGVEVHNAKTKPREEQYNSTYRVVSVLTVLHQDWLNGKEYKCKVSNKALPAPIEKTISKAKGQPREPQVYTLPPSREEMTKNQVSLTCLVKGFYPSDIAVEWESNGQPENNYKTTPPVLDSDGSFFLYSKLTVDKSRWQQGNVFSCSVMHEALHNHYTQKSLSLSPGK

SEQ ID NO: 80 - DNA, 2013 bp, Homo
caggtgcagctgcaggaatctggcccaggcctggtgaagccttctgagacactgtctttgacctgtacagtgtctggcttttctctgtcttcttatgatatttcctggattagacagcctcctggcaagggcctggagtggctgggagtgatttggacaggaggcggaacaaattataactctgcttttatgtctaggctgaccatctctaaggataatagtaaatctcaggtgtctctgaagctgtcttctgtgaccgctgctgatacagccgtgtactattgtgttagaatggattattggggccagggcacactggtgaccgtgtcttctgcaagtaccaagggacctagtgttttccctcttgcaccttgctccaggtcaacatcagagtccacagctgctcttggatgtctcgttaaggactacttcccagagccagttaccgtatcctggaactccggagctttgacaagcggcgttcatacattcccagctgtgttgcagagttctgggttgtacagtttgagctcagtggtgaccgtgccttcatcttctttgggcactaagacctacacctgcaacgtggatcacaagccaagcaacaccaaggtggataagagggtgggtggaggcggttcaggcggaggtggcagcggaggtggcgggagtcaagttcagctggtgcagagcggagctgaggtgaagaagcccggcgccagcgtgaaggtgagctgtaagggcagcggctacaccttcaccgactacgccatccactgggtgagacaagctcccggtcagtctttagaatggatcggcgtgttcagcatctactacgagaacatcaactataaccagaagttcaagggtcgtgccaccatgaccgtggacaagagcaccagcaccgcctacatggagctgaggtctttaaggagcgacgacaccgccgtgtactactgcgctcgtagggacggcggcaccatcaactactggggccaaggtactttagtgacagtgagcagcgcgagcaccaagggaccttccgtgtttcccctcgcccccagctccaaaagcaccagcggcggaacagctgctctcggctgtctcgtcaaggattacttccccgagcccgtgaccgtgagctggaacagcggagccctgacaagcggcgtccacaccttccctgctgtcctacagtcctccggactgtacagcctgagcagcgtggtgacagtccctagcagctccctgggcacccagacatatatttgcaacgtgaatcacaagcccagcaacaccaaggtcgataagaaggtggagcctaagtcctgcgacaagacccacacatgtcccccctgtcccgctcctgaagctgctggaggcccttccgtgttcctgttcccccctaagcccaaggacaccctgatgatttccaggacacccgaggtgacctgtgtggtggtggacgtcagccacgaggaccccgaggtgaaattcaactggtacgtcgatggcgtggaggtgcacaacgctaagaccaagcccagggaggagcagtacaattccacctacagggtggtgtccgtgctgaccgtcctccatcaggactggctgaacggcaaagagtataagtgcaaggtgagcaacaaggccctccctgctcccatcgagaagaccatcagcaaagccaagggccagcccagggaacctcaagtctataccctgcctcccagcagggaggagatgaccaagaaccaagtgagcctcacatgcctcgtcaagggcttctatccttccgatattgccgtcgagtgggagtccaacggacagcccgagaacaactacaagacaacaccccccgtgctcgattccgatggcagcttcttcctgtactccaagctgaccgtggacaagtccagatggcaacaaggcaacgtcttcagttgcagcgtcatgcatgaggccctccacaaccactacacccagaagagcctctccctgagccctggaaag

SEQ ID NO: 81 - protein, 671 aa, Homo
QVQLVQSGAEVKKPGASVKVSCKGSGYTFTDYAIHWVRQAPGQSLEWIGVFSIYYENINYNQKFKGRATMTVDKSTSTAYMELRSLRSDDTAVYYCARRDGGTINYWGQGTLVTVSSASTKGPSVFPLAPCSRSTSESTAALGCLVKDYFPEPVTVSWNSGALTSGVHTFPAVLQSSGLYSLSSVVTVPSSSLGTKTYTCNVDHKPSNTKVDKRVGGGGSGGGGSGGGGSQVQLQESGPGLVKPSETLSLTCTVSGFSLSSYDISWIRQPPGKGLEWLGVIWTGGGTNYNSAFMSRLTISKDNSKSQVSLKLSSVTAADTAVYYCVRMDYWGQGTLVTVSSASTKGPSVFPLAPSSKSTSGGTAALGCLVKDYFPEPVTVSWNSGALTSGVHTFPAVLQSSGLYSLSSVVTVPSSSLGTQTYICNVNHKPSNTKVDKKVEPKSCDKTHTCPPCPAPEAAGGPSVFLFPPKPKDTLMISRTPEVTCVVVDVSHEDPEVKFNWYVDGVEVHNAKTKPREEQYNSTYRVVSVLTVLHQDWLNGKEYKCKVSNKALPAPIEKTISKAKGQPREPQVYTLPPSREEMTKNQVSLTCLVKGFYPSDIAVEWESNGQPENNYKTTPPVLDSDGSFFLYSKLTVDKSRWQQGNVFSCSVMHEALHNHYTQKSLSLSPGK

SEQ ID NO: 82 - DNA, 2013 bp, Homo
caagttcagctggtgcagagcggagctgaggtgaagaagcccggcgccagcgtgaaggtgagctgtaagggcagcggctacaccttcaccgactacgccatccactgggtgagacaagctcccggtcagtctttagaatggatcggcgtgttcagcatctactacgagaacatcaactataaccagaagttcaagggtcgtgccaccatgaccgtggacaagagcaccagcaccgcctacatggagctgaggtctttaaggagcgacgacaccgccgtgtactactgcgctcgtagggacggcggcaccatcaactactggggccaaggtactttagtgacagtgagcagcgcaagtaccaagggacctagtgttttccctcttgcaccttgctccaggtcaacatcagagtccacagctgctcttggatgtctcgttaaggactacttcccagagccagttaccgtatcctggaactccggagctttgacaagcggcgttcatacattcccagctgtgttgcagagttctgggttgtacagtttgagctcagtggtgaccgtgccttcatcttctttgggcactaagacctacacctgcaacgtggatcacaagccaagcaacaccaaggtggataagagggtgggtggaggcggttcaggcggaggtggcagcggaggtggcgggagtcaggtgcagctgcaggaatctggcccaggcctggtgaagccttctgagacactgtctttgacctgtacagtgtctggcttttctctgtcttcttatgatatttcctggattagacagcctcctggcaagggcctggagtggctgggagtgatttggacaggaggcggaacaaattataactctgcttttatgtctaggctgaccatctctaaggataatagtaaatctcaggtgtctctgaagctgtcttctgtgaccgctgctgatacagccgtgtactattgtgttagaatggattattggggccagggcacactggtgaccgtgtcttctgcgagcaccaagggaccttccgtgtttcccctcgcccccagctccaaaagcaccagcggcggaacagctgctctcggctgtctcgtcaaggattacttccccgagcccgtgaccgtgagctggaacagcggagccctgacaagcggcgtccacaccttccctgctgtcctacagtcctccggactgtacagcctgagcagcgtggtgacagtccctagcagctccctgggcacccagacatatatttgcaacgtgaatcacaagcccagcaacaccaaggtcgataagaaggtggagcctaagtcctgcgacaagacccacacatgtcccccctgtcccgctcctgaagctgctggaggcccttccgtgttcctgttcccccctaagcccaaggacaccctgatgatttccaggacacccgaggtgacctgtgtggtggtggacgtcagccacgaggaccccgaggtgaaattcaactggtacgtcgatggcgtggaggtgcacaacgctaagaccaagcccagggaggagcagtacaattccacctacagggtggtgtccgtgctgaccgtcctccatcaggactggctgaacggcaaagagtataagtgcaaggtgagcaacaaggccctccctgctcccatcgagaagaccatcagcaaagccaagggccagcccagggaacctcaagtctataccctgcctcccagcagggaggagatgaccaagaaccaagtgagcctcacatgcctcgtcaagggcttctatccttccgatattgccgtcgagtgggagtccaacggacagcccgagaacaactacaagacaacaccccccgtgctcgattccgatggcagcttcttcctgtactccaagctgaccgtggacaagtccagatggcaacaaggcaacgtcttcagttgcagcgtcatgcatgaggccctccacaaccactacacccagaagagcctctccctgagccctggaaag

SEQ ID NO: 83 - protein, 117 aa, Homo
EVKLVESGGGLVQPGGSLRLSCAASGFAFSSYDMSWVRQAPGKRLEWVATISGGGRYTYYPDTVKGRFTISRDNAKNSHYLQMNSLRAEDTAVYFCASPYGGYFDVWGQGTLVTVSS

SEQ ID NO: 84 - protein, 107 aa, Homo
EIVLTQSPATLSLSPGERATLSCRASQSISNFLHWYQQKPGQAPRLLIKYASQSISGIPARFSGSGSGTDFTLTISSLEPEDFAVYFCQQSNSWPHTFGQGTKVEIK

SEQ ID NO: 85 - protein, 5 aa, Mus musculus
SYWMH

SEQ ID NO: 86 - protein, 17 aa, Mus musculus
EINPGNGHTNYNEKFKS

SEQ ID NO: 87 - protein, 10 aa, Mus musculus
SFTTARGFAY

SEQ ID NO: 88 - protein, 11 aa, Mus musculus
RASQTISDYLH

SEQ ID NO: 89 - protein, 7 aa, Mus musculus
YASQSIS

SEQ ID NO: 90 - protein, 9 aa, Mus musculus
QDGHSFPPT

SEQ ID NO: 91 - protein, 119 aa, Homo
QVQLVQSGAEVKKPGASVKVSCKASGYTFSSYWMHWVRQAPGQGLEWMGEINPGNGHTNYNEKFKSRVTLTVDKSTSTVYMELSSLRSEDTAVYYCARSFTTARGFAYWGQGTLVTVSS

SEQ ID NO: 92 - protein, 107 aa, Homo
EIVMTQSPDFQSVTPKEKVTITCRASQTISDYLHWYQQKPDQSPKLLIKYASQSISGIPSRFSGSGSGSDFTLTINSLEAEDAATYYCQDGHSFPPTFGQGTKVEIK

SEQ ID NO: 93 - protein, 214 aa, Homo
EIVMTQSPDFQSVTPKEKVTITCRASQTISDYLHWYQQKPDQSPKLLIKYASQSISGIPSRFSGSGSGSDFTLTINSLEAEDAATYYCQDGHSFPPTFGQGTKVEIKRTVAAPSVFIFPPSDEQLKSGTASVVCLLNNFYPREAKVQWKVDNALQSGNSQESVTEQDSKDSTYSLSSTLTLSKADYEKHKVYACEVTHQGLSSPVTKSFNRGEC

SEQ ID NO: 94 - DNA, 642 bp, Homo
gagatcgtgatgacccagtctcctgattttcagtctgtgacccctaaggagaaggtgacaatcacctgtagagcttctcagaccatctctgattatctgcattggtatcagcagaagcctgatcagtctcctaagctgctgatcaagtatgcttctcagtctatctctggcattccttctaggttttccggctctggctctggctctgattttacactgaccatcaattctctggaggctgaggatgctgccacctattattgtcaggacggccactcttttcctcctacctttggccagggaaccaaggtggagatcaagagaaccgtcgccgctcccagcgtcttcatcttcccccccagcgatgagcagctgaagagcggaaccgccagcgtggtgtgcctgctgaacaacttctaccccagggaggccaaggtgcaatggaaggtggacaacgccctacagagcggcaactcccaggagagcgtgaccgagcaggacagcaaggatagcacctacagcctgagcagcaccctcaccctgagcaaggccgactacgagaagcacaaggtgtacgcctgcgaggtgacccatcagggcctgagcagccctgtgaccaagagcttcaacaggggcgagtgc

SEQ ID NO: 95 - protein, 676 aa, Homo
EVKLVESGGGLVQPGGSLRLSCAASGFAFSSYDMSWVRQAPGKRLEWVATISGGGRYTYYPDTVKGRFTISRDNAKNSHYLQMNSLRAEDTAVYFCASPYGGYFDVWGQGTLVTVSSASTKGPSVFPLAPCSRSTSESTAALGCLVKDYFPEPVTVSWNSGALTSGVHTFPAVLQSSGLYSLSSVVTVPSSSLGTKTYTCNVDHKPSNTKVDKRVGGGGSGGGGSGGGGSQVQLVQSGAEVKKPGASVKVSCKASGYTFSSYWMHWVRQAPGQGLEWMGEINPGNGHTNYNEKFKSRVTLTVDKSTSTVYMELSSLRSEDTAVYYCARSFTTARGFAYWGQGTLVTVSSASTKGPSVFPLAPCSRSTSESTAALGCLVKDYFPEPVTVSWNSGALTSGVHTFPAVLQSSGLYSLSSVVTVPSSSLGTKTYTCNVDHKPSNTKVDKRVESKYGPPCPPCPAPEFLGGPSVFLFPPKPKDTLMISRTPEVTCVVVDVSQEDPEVQFNWYVDGVEVHNAKTKPREEQFNSTYRVVSVLTVLHQDWLNGKEYKCKVSNKGLPSSIEKTISKAKGQPREPQVYTLPPSQEEMTKNQVSLTCLVKGFYPSDIAVEWESNGQPENNYKTTPPVLDSDGSFFLYSRLTVDKSRWQEGNVFSCSVMHEALHNHYTQKSLSLSLGK

SEQ ID NO: 96 - DNA, 2028 bp, Homo
gaggtcaagctggtggaaagcggcggcggcctggtgcagcctggaggatccctgcggctgagctgcgctgcctccggcttcgctttcagctcctatgacatgtcctgggtgaggcaggcccctggaaagaggctggagtgggtggctaccatctccggaggcggaaggtacacctactaccccgacacagtgaagggaaggttcaccatcagccgggataacgccaaaaacagccactatctccagatgaactccctgagggccgaagatacagccgtgtatttctgtgcctccccctacggaggctattttgacgtgtggggacagggcaccctggtgaccgtctcctccgcaagtaccaagggacctagtgttttccctcttgcaccttgctccaggtcaacatcagagtccacagctgctcttggatgtctcgttaaggactacttcccagagccagttaccgtatcctggaactccggagctttgacaagcggcgttcatacattcccagctgtgttgcagagttctgggttgtacagtttgagctcagtggtgaccgtgccttcatcttctttgggcactaagacctacacctgcaacgtggatcacaagccaagcaacaccaaggtggataagagggtgggtggaggcggttcaggcggaggtggcagcggaggtggcgggagtcaggtgcagctggtgcagagcggcgctgaagtgaagaagccaggcgcttctgtaaaggtgtcttgtaaggcttctggctatacattttcttcttattggatgcactgggtgagacaggctcctggccagggactggagtggatgggtgagatcaatcctggcaatggccatactaactacaacgagaagttcaagtccagggtgaccctgaccgtggacaagtccacctccaccgtgtacatggagctgagctccctgaggtccgaggacaccgccgtgtactactgcgcccggagcttcactaccgcccgcggcttcgcctattggggccagggcaccctggtgaccgtgagctccgcctccaccaagggcccatcggtcttccccctggcaccctgctccaggagcacctctgagtccacagcggccctgggctgcctggtcaaggactacttccccgaaccggtgacggtgtcgtggaactcaggcgccctgaccagcggcgtgcacaccttcccggctgtcctacagtcctcaggactctactccctcagcagcgtggtgaccgtgccctccagcagcttgggcaccaagacatatacctgtaatgtggatcacaagccttccaatacaaaagtggacaagagagttgagtccaagtacggcccaccatgtcctccatgtccagcccctgaatttttgggcgggccttctgtctttctgtttcctcctaaacctaaagataccctgatgatcagccgcacacccgaagtcacttgtgtggtcgtggatgtgtctcaggaagatcccgaagtgcagtttaactggtatgtcgatggcgtggaagtgcataatgccaaaactaagccccgcgaagaacagttcaacagcacttatcgggtcgtgtctgtgctcacagtcctccatcaggattggctgaatgggaaagaatataagtgcaaggtgagcaataagggcctccccagcagcatcgagaagactattagcaaagccaaagggcagccacgggaaccccaggtgtacactctgcccccctctcaggaggagatgactaaaaatcaggtctctctgacttgtctggtgaaagggttttatcccagcgacattgccgtggagtgggagtctaatggccagcccgagaataattataagacaactccccccgtcctggactctgacggcagctttttcctgtattctcggctgacagtggacaaaagtcgctggcaggagggcaatgtctttagttgcagtgtcatgcatgaggccctgcacaatcactatacacagaaaagcctgtctctgagtctgggcaaa

SEQ ID NO: 97 - protein, 676 aa, Homo
QVQLVQSGAEVKKPGASVKVSCKASGYTFSSYWMHWVRQAPGQGLEWMGEINPGNGHTNYNEKFKSRVTLTVDKSTSTVYMELSSLRSEDTAVYYCARSFTTARGFAYWGQGTLVTVSSASTKGPSVFPLAPCSRSTSESTAALGCLVKDYFPEPVTVSWNSGALTSGVHTFPAVLQSSGLYSLSSVVTVPSSSLGTKTYTCNVDHKPSNTKVDKRVGGGGSGGGGSGGGGSEVKLVESGGGLVQPGGSLRLSCAASGFAFSSYDMSWVRQAPGKRLEWVATISGGGRYTYYPDTVKGRFTISRDNAKNSHYLQMNSLRAEDTAVYFCASPYGGYFDVWGQGTLVTVSSASTKGPSVFPLAPCSRSTSESTAALGCLVKDYFPEPVTVSWNSGALTSGVHTFPAVLQSSGLYSLSSVVTVPSSSLGTKTYTCNVDHKPSNTKVDKRVESKYGPPCPPCPAPEFLGGPSVFLFPPKPKDTLMISRTPEVTCVVVDVSQEDPEVQFNWYVDGVEVHNAKTKPREEQFNSTYRVVSVLTVLHQDWLNGKEYKCKVSNKGLPSSIEKTISKAKGQPREPQVYTLPPSQEEMTKNQVSLTCLVKGFYPSDIAVEWESNGQPENNYKTTPPVLDSDGSFFLYSRLTVDKSRWQEGNVFSCSVMHEALHNHYTQKSLSLSLGK

SEQ ID NO: 98 - DNA, 2028 bp, Homo
caggtgcagctggtgcagagcggcgctgaagtgaagaagccaggcgcttctgtaaaggtgtcttgtaaggcttctggctatacattttcttcttattggatgcactgggtgagacaggctcctggccagggactggagtggatgggtgagatcaatcctggcaatggccatactaactacaacgagaagttcaagtccagggtgaccctgaccgtggacaagtccacctccaccgtgtacatggagctgagctccctgaggtccgaggacaccgccgtgtactactgcgcccggagcttcactaccgcccgcggcttcgcctattggggccagggcaccctggtgaccgtgagctccgcaagtaccaagggacctagtgttttccctcttgcaccttgctccaggtcaacatcagagtccacagctgctcttggatgtctcgttaaggactacttcccagagccagttaccgtatcctggaactccggagctttgacaagcggcgttcatacattcccagctgtgttgcagagttctgggttgtacagtttgagctcagtggtgaccgtgccttcatcttctttgggcactaagacctacacctgcaacgtggatcacaagccaagcaacaccaaggtggataagagggtgggtggaggcggttcaggcggaggtggcagcggaggtggcgggagtgaggtcaagctggtggaaagcggcggcggcctggtgcagcctggaggatccctgcggctgagctgcgctgcctccggcttcgctttcagctcctatgacatgtcctgggtgaggcaggcccctggaaagaggctggagtgggtggctaccatctccggaggcggaaggtacacctactaccccgacacagtgaagggaaggttcaccatcagccgggataacgccaaaaacagccactatctccagatgaactccctgagggccgaagatacagccgtgtatttctgtgcctccccctacggaggctattttgacgtgtggggacagggcaccctggtgaccgtctcctccgcctccaccaagggcccatcggtcttccccctggcaccctgctccaggagcacctctgagtccacagcggccctgggctgcctggtcaaggactacttccccgaaccggtgacggtgtcgtggaactcaggcgccctgaccagcggcgtgcacaccttcccggctgtcctacagtcctcaggactctactccctcagcagcgtggtgaccgtgccctccagcagcttgggcaccaagacatatacctgtaatgtggatcacaagccttccaatacaaaagtggacaagagagttgagtccaagtacggcccaccatgtcctccatgtccagcccctgaatttttgggcgggccttctgtctttctgtttcctcctaaacctaaagataccctgatgatcagccgcacacccgaagtcacttgtgtggtcgtggatgtgtctcaggaagatcccgaagtgcagtttaactggtatgtcgatggcgtggaagtgcataatgccaaaactaagccccgcgaagaacagttcaacagcacttatcgggtcgtgtctgtgctcacagtcctccatcaggattggctgaatgggaaagaatataagtgcaaggtgagcaataagggcctccccagcagcatcgagaagactattagcaaagccaaagggcagccacgggaaccccaggtgtacactctgcccccctctcaggaggagatgactaaaaatcaggtctctctgacttgtctggtgaaagggttttatcccagcgacattgccgtggagtgggagtctaatggccagcccgagaataattataagacaactccccccgtcctggactctgacggcagctttttcctgtattctcggctgacagtggacaaaagtcgctggcaggagggcaatgtctttagttgcagtgtcatgcatgaggccctgcacaatcactatacacagaaaagcctgtctctgagtctgggcaaa

SEQ ID NO: 99 - protein, 5 aa, Mus musculus
TTGMQ

SEQ ID NO: 100 - protein, 17 aa, Mus musculus
WINTHSGVPKYVEDFKG

SEQ ID NO: 101 - protein, 13 aa, Mus musculus
SGNGNYDLAYFAY

SEQ ID NO: 102 - protein, 11 aa, Mus musculus
RASQSISDYLH

SEQ ID NO: 103 - protein, 7 aa, Mus musculus
YASHSIS

SEQ ID NO: 104 - protein, 9 aa, Mus musculus
QHGHSFPWT

SEQ ID NO: 105 - protein, 122 aa, Homo
QIQLVQSGSELKKPGASVKVSCKASGYAFTTTGMQWVREAPGQGLEWIGWINTHSGVPKYVEDFKGRFVFSLDTSVNTAYLQISSLKAEDTAVYYCVRSGNGNYDLAYFAYWGQGTLVTVSS

SEQ ID NO: 106 - protein, 107 aa, Homo
EIVLTQSPATLSLSPGERATLSCRASQSISDYLHWYQQKPGQSPRLLIKYASHSISGIPARFSGSGSGSDFTLTISSLEPEDFAVYYCQHGHSFPWTFGQGTKVEIK

SEQ ID NO: 107 - protein, 214 aa, Homo
EIVLTQSPATLSLSPGERATLSCRASQSISDYLHWYQQKPGQSPRLLIKYASHSISGIPARFSGSGSGSDFTLTISSLEPEDFAVYYCQHGHSFPWTFGQGTKVEIKRTVAAPSVFIFPPSDEQLKSGTASVVCLLNNFYPREAKVQWKVDNALQSGNSQESVTEQDSKDSTYSLSSTLTLSKADYEKHKVYACEVTHQGLSSPVTKSFNRGEC

SEQ ID NO: 108 - DNA, 642 bp, Homo
gaaatcgtgctgacacagtctcctgctacactgtctctgagtcctggagaaagagctacactgtcttgtagagcttcccagtctatctccgattatctgcactggtaccagcagaagcctggccagtctcctagactgctgatcaagtatgcttctcattctatttctggcatcccagctaggtttagtggatctggctctggaagcgactttacactgaccatttcttctctggagcctgaggattttgctgtgtattactgtcagcacggccattcttttccttggacctttggccagggcacaaaggtggagatcaagagaaccgtcgccgctcccagcgtcttcatcttcccccccagcgatgagcagctgaagagcggaaccgccagcgtggtgtgcctgctgaacaacttctaccccagggaggccaaggtgcaatggaaggtggacaacgccctacagagcggcaactcccaggagagcgtgaccgagcaggacagcaaggatagcacctacagcctgagcagcaccctcaccctgagcaaggccgactacgagaagcacaaggtgtacgcctgcgaggtgacccatcagggcctgagcagccctgtgaccaagagcttcaacaggggcgagtgc

SEQ ID NO: 109 - protein, 679 aa, Homo
EVKLVESGGGLVQPGGSLRLSCAASGFAFSSYDMSWVRQAPGKRLEWVATISGGGRYTYYPDTVKGRFTISRDNAKNSHYLQMNSLRAEDTAVYFCASPYGGYFDVWGQGTLVTVSSASTKGPSVFPLAPCSRSTSESTAALGCLVKDYFPEPVTVSWNSGALTSGVHTFPAVLQSSGLYSLSSVVTVPSSSLGTKTYTCNVDHKPSNTKVDKRVGGGGSGGGGSGGGGSQIQLVQSGSELKKPGASVKVSCKASGYAFTTTGMQWVREAPGQGLEWIGWINTHSGVPKYVEDFKGRFVFSLDTSVNTAYLQISSLKAEDTAVYYCVRSGNGNYDLAYFAYWGQGTLVTVSSASTKGPSVFPLAPCSRSTSESTAALGCLVKDYFPEPVTVSWNSGALTSGVHTFPAVLQSSGLYSLSSVVTVPSSSLGTKTYTCNVDHKPSNTKVDKRVESKYGPPCPPCPAPEFLGGPSVFLFPPKPKDTLMISRTPEVTCVVVDVSQEDPEVQFNWYVDGVEVHNAKTKPREEQFNSTYRVVSVLTVLHQDWLNGKEYKCKVSNKGLPSSIEKTISKAKGQPREPQVYTLPPSQEEMTKNQVSLTCLVKGFYPSDIAVEWESNGQPENNYKTTPPVLDSDGSFFLYSRLTVDKSRWQEGNVFSCSVMHEALHNHYTQKSLSLSLGK

SEQ ID NO: 110 - DNA, 2037 bp, Homo
gaggtcaagctggtggaaagcggcggcggcctggtgcagcctggaggatccctgcggctgagctgcgctgcctccggcttcgctttcagctcctatgacatgtcctgggtgaggcaggcccctggaaagaggctggagtgggtggctaccatctccggaggcggaaggtacacctactaccccgacacagtgaagggaaggttcaccatcagccgggataacgccaaaaacagccactatctccagatgaactccctgagggccgaagatacagccgtgtatttctgtgcctccccctacggaggctattttgacgtgtggggacagggcaccctggtgaccgtctcctccgcaagtaccaagggacctagtgttttccctcttgcaccttgctccaggtcaacatcagagtccacagctgctcttggatgtctcgttaaggactacttcccagagccagttaccgtatcctggaactccggagctttgacaagcggcgttcatacattcccagctgtgttgcagagttctgggttgtacagtttgagctcagtggtgaccgtgccttcatcttctttgggcactaagacctacacctgcaacgtggatcacaagccaagcaacaccaaggtggataagagggtgggtggaggcggttcaggcggaggtggcagcggaggtggcgggagtcagatccagctggtgcagtccggctccgagctgaagaagcccggcgcctccgtcaaggtgtcctgcaaggccagtggctacgcctttaccaccaccggcatgcagtgggtgagggaggccccaggccagggcctggagtggatcggctggatcaacacacattctggagtgcctaagtatgtggaagactttaagggcagattcgtgttttctctggatacctctgtgaataccgcttacctgcagatttcttctctgaaggctgaggacacagctgtgtattactgtgtgagatctggaaatggaaactatgatctggcttattttgcctattggggccagggcacactggtgaccgtgtcttctgcctccaccaagggcccatcggtcttccccctggcaccctgctccaggagcacctctgagtccacagcggccctgggctgcctggtcaaggactacttccccgaaccggtgacggtgtcgtggaactcaggcgccctgaccagcggcgtgcacaccttcccggctgtcctacagtcctcaggactctactccctcagcagcgtggtgaccgtgccctccagcagcttgggcaccaagacatatacctgtaatgtggatcacaagccttccaatacaaaagtggacaagagagttgagtccaagtacggcccaccatgtcctccatgtccagcccctgaatttttgggcgggccttctgtctttctgtttcctcctaaacctaaagataccctgatgatcagccgcacacccgaagtcacttgtgtggtcgtggatgtgtctcaggaagatcccgaagtgcagtttaactggtatgtcgatggcgtggaagtgcataatgccaaaactaagccccgcgaagaacagttcaacagcacttatcgggtcgtgtctgtgctcacagtcctccatcaggattggctgaatgggaaagaatataagtgcaaggtgagcaataagggcctccccagcagcatcgagaagactattagcaaagccaaagggcagccacgggaaccccaggtgtacactctgcccccctctcaggaggagatgactaaaaatcaggtctctctgacttgtctggtgaaagggttttatcccagcgacattgccgtggagtgggagtctaatggccagcccgagaataattataagacaactccccccgtcctggactctgacggcagctttttcctgtattctcggctgacagtggacaaaagtcgctggcaggagggcaatgtctttagttgcagtgtcatgcatgaggccctgcacaatcactatacacagaaaagcctgtctctgagtctgggcaaa

SEQ ID NO: 111 - protein, 679 aa, Homo
QIQLVQSGSELKKPGASVKVSCKASGYAFTTTGMQWVREAPGQGLEWIGWINTHSGVPKYVEDFKGRFVFSLDTSVNTAYLQISSLKAEDTAVYYCVRSGNGNYDLAYFAYWGQGTLVTVSSASTKGPSVFPLAPCSRSTSESTAALGCLVKDYFPEPVTVSWNSGALTSGVHTFPAVLQSSGLYSLSSVVTVPSSSLGTKTYTCNVDHKPSNTKVDKRVGGGGSGGGGSGGGGSEVKLVESGGGLVQPGGSLRLSCAASGFAFSSYDMSWVRQAPGKRLEWVATISGGGRYTYYPDTVKGRFTISRDNAKNSHYLQMNSLRAEDTAVYFCASPYGGYFDVWGQGTLVTVSSASTKGPSVFPLAPCSRSTSESTAALGCLVKDYFPEPVTVSWNSGALTSGVHTFPAVLQSSGLYSLSSVVTVPSSSLGTKTYTCNVDHKPSNTKVDKRVESKYGPPCPPCPAPEFLGGPSVFLFPPKPKDTLMISRTPEVTCVVVDVSQEDPEVQFNWYVDGVEVHNAKTKPREEQFNSTYRVVSVLTVLHQDWLNGKEYKCKVSNKGLPSSIEKTISKAKGQPREPQVYTLPPSQEEMTKNQVSLTCLVKGFYPSDIAVEWESNGQPENNYKTTPPVLDSDGSFFLYSRLTVDKSRWQEGNVFSCSVMHEALHNHYTQKSLSLSLGK

SEQ ID NO: 112 - DNA, 2037 bp, Homo
cagatccagctggtgcagtccggctccgagctgaagaagcccggcgcctccgtcaaggtgtcctgcaaggccagtggctacgcctttaccaccaccggcatgcagtgggtgagggaggccccaggccagggcctggagtggatcggctggatcaacacacattctggagtgcctaagtatgtggaagactttaagggcagattcgtgttttctctggatacctctgtgaataccgcttacctgcagatttcttctctgaaggctgaggacacagctgtgtattactgtgtgagatctggaaatggaaactatgatctggcttattttgcctattggggccagggcacactggtgaccgtgtcttctgcaagtaccaagggacctagtgttttccctcttgcaccttgctccaggtcaacatcagagtccacagctgctcttggatgtctcgttaaggactacttcccagagccagttaccgtatcctggaactccggagctttgacaagcggcgttcatacattcccagctgtgttgcagagttctgggttgtacagtttgagctcagtggtgaccgtgccttcatcttctttgggcactaagacctacacctgcaacgtggatcacaagccaagcaacaccaaggtggataagagggtgggtggaggcggttcaggcggaggtggcagcggaggtggcgggagtgaggtcaagctggtggaaagcggcggcggcctggtgcagcctggaggatccctgcggctgagctgcgctgcctccggcttcgctttcagctcctatgacatgtcctgggtgaggcaggcccctggaaagaggctggagtgggtggctaccatctccggaggcggaaggtacacctactaccccgacacagtgaagggaaggttcaccatcagccgggataacgccaaaaacagccactatctccagatgaactccctgagggccgaagatacagccgtgtatttctgtgcctccccctacggaggctattttgacgtgtggggacagggcaccctggtgaccgtctcctccgcctccaccaagggcccatcggtcttccccctggcaccctgctccaggagcacctctgagtccacagcggccctgggctgcctggtcaaggactacttccccgaaccggtgacggtgtcgtggaactcaggcgccctgaccagcggcgtgcacaccttcccggctgtcctacagtcctcaggactctactccctcagcagcgtggtgaccgtgccctccagcagcttgggcaccaagacatatacctgtaatgtggatcacaagccttccaatacaaaagtggacaagagagttgagtccaagtacggcccaccatgtcctccatgtccagcccctgaatttttgggcgggccttctgtctttctgtttcctcctaaacctaaagataccctgatgatcagccgcacacccgaagtcacttgtgtggtcgtggatgtgtctcaggaagatcccgaagtgcagtttaactggtatgtcgatggcgtggaagtgcataatgccaaaactaagccccgcgaagaacagttcaacagcacttatcgggtcgtgtctgtgctcacagtcctccatcaggattggctgaatgggaaagaatataagtgcaaggtgagcaataagggcctccccagcagcatcgagaagactattagcaaagccaaagggcagccacgggaaccccaggtgtacactctgcccccctctcaggaggagatgactaaaaatcaggtctctctgacttgtctggtgaaagggttttatcccagcgacattgccgtggagtgggagtctaatggccagcccgagaataattataagacaactccccccgtcctggactctgacggcagctttttcctgtattctcggctgacagtggacaaaagtcgctggcaggagggcaatgtctttagttgcagtgtcatgcatgaggccctgcacaatcactatacacagaaaagcctgtctctgagtctgggcaaa

SEQ ID NO: 113 - protein, 119 aa, Homo
QVQLKQSGPGLVQPSQSLSITCTVSGFSLTNYGVHWVRQSPGKGLEWLGVIWSGGNTDYNTPFTSRLSINKDNSKSQVFFKMNSLQSNDTAIYYCARALTYYDYEFAYWGQGTLVTVSA

SEQ ID NO: 114 - protein, 107 aa, Homo
DILLTQSPVILSVSPGERVSFSCRASQSIGTNIHWYQQRTNGSPRLLIKYASESISGIPSRFSGSGSGTDFTLSINSVESEDIADYYCQQNNNWPTTFGAGTKLELK

SEQ ID NO: 115 - protein, 120 aa, Homo [sequence omitted]

SEQ ID NO: 116 - protein, 107 aa, Homo [sequence omitted]

SEQ ID NO: 117 - protein, 119 aa, Homo [sequence omitted]

SEQ ID NO: 118 - protein, 107 aa, Homo [sequence omitted]

SEQ ID NO: 119 - protein, 118 aa, Homo
QVQLVESGGGVVQPGRSLRLSCAASGFTFSSYTMHWVRQAPGKGLEWVTFISYDGNNKYYADSVKGRFTISRDNSKNTLYLQMNSLRAEDTAIYYCARTGWLGPFDYWGQGTLVTVSS

SEQ ID NO: 120 - protein, 108 aa, Homo
EIVLTQSPGTLSLSPGERATLSCRASQSVGSSYLAWYQQKPGQAPRLLIYGAFSRATGIPDRFSGSGSGTDFTLTISRLEPEDFAVYYCQQYGSSPWTFGQGTKVEIK

SEQ ID NO: 121 - protein, 116 aa, Homo
EVQLVESGGGLVKPGGSLRLSCAASGFTFSDDYMAWFRQAPGKRLEWVASISHGGDYIYYADNLKGRFTISRDNAKNSLYLQMNSLRAEDTAVYFCSRDRRSIDYWGQGTLVTVSS

SEQ ID NO: 122 - protein, 107 aa, Homo
DIQMTQSPSSLSASVGDRVTITCRASQDISNYLSWYQQKPGKTIKLLIYYTSRLHSGVPSRFSGSGSGTDYTFTISSLQPEDIATYFCQQGKTLPYTFGQGTKVEIK

SEQ ID NO: 123 - protein, 214 aa, Homo
DILLTQSPVILSVSPGERVSFSCRASQSIGTNIHWYQQRTNGSPRLLIKYASESISGIPSRFSGSGSGTDFTLSINSVESEDIADYYCQQNNNWPTTFGAGTKLELKRTVAAPSVFIFPPSDEQLKSGTASVVCLLNNFYPREAKVQWKVDNALQSGNSQESVTEQDSKDSTYSLSSTLTLSKADYEKHKVYACEVTHQGLSSPVTKSFNRGEC

SEQ ID NO: 124 - DNA, 642 bp, Homo
gacatcctgctgacccagtcccccgtgatcctgtccgtgtcccctggcgagagggtgtccttctcctgcagggcctcccagtccatcggcaccaacatccactggtaccagcagaggaccaacggctcccccaggctgctgatcaagtacgcctccgagagcatcagcggcatcccctccaggttttccggctccggctccggaaccgacttcaccctgtccatcaactccgtggagtccgaggacatcgccgactactactgccagcagaacaacaactggcccaccacctttggcgccggcaccaagctggagctgaagaggaccgtggccgccccctccgtgttcatttttccccctagcgacgagcagctgaagagcggcaccgctagcgtggtgtgcctgctgaacaacttctaccccagggaggccaaggtgcagtggaaagtggacaacgccctgcagagcggcaactcccaggagtccgtgaccgagcaggacagcaaggacagcacctactccctgtcctccaccctgaccctgtccaaggccgactacgagaagcacaaggtgtacgcctgtgaggtgacacaccagggcctgtcctcccccgtgacaaagtccttcaacaggggcgagtgc

SEQ ID NO: 125 - protein, 214 aa, Homo
DIQMTQSPSSLSASVGDRVTITCKASQDVSIGVAWYQQKPGKAPKLLIYSASYRYTGVPSRFSGSGSGTDFTLTISSLQPEDFATYYCQQYYIYPYTFGQGTKVEIKRTVAAPSVFIFPPSDEQLKSGTASVVCLLNNFYPREAKVQWKVDNALQSGNSQESVTEQDSKDSTYSLSSTLTLSKADYEKHKVYACEVTHQGLSSPVTKSFNRGEC

SEQ ID NO: 126 - DNA, 642 bp, Homo
gacatccagatgacccagtctccttcttctctgtctgcttctgtgggcgatagagtgaccatcacctgtaaggcttctcaggatgtgtctatcggcgtggcctggtatcagcagaagcctggaaaggctcctaagctgctgatctactctgcttcttacagatatactggcgtgccttctagattttctggctctggctctggcacagattttacactgaccatctcttctctgcagcctgaggacttcgctacctattactgtcagcagtactacatctatccttatacctttggccagggcaccaaggtggagatcaagagaaccgtcgccgctcccagcgtcttcatcttcccccccagcgatgagcagctgaagagcggaaccgccagcgtggtgtgcctgctgaacaacttctaccccagggaggccaaggtgcaatggaaggtggacaacgccctacagagcggcaactcccaggagagcgtgaccgagcaggacagcaaggatagcacctacagcctgagcagcaccctcaccctgagcaaggccgactacgagaagcacaaggtgtacgcctgcgaggtgacccatcagggcctgagcagccctgtgaccaagagcttcaacaggggcgagtgc

SEQ ID NO: 127 - protein, 215 aa, Homo
EIVLTQSPGTLSLSPGERATLSCRASQSVGSSYLAWYQQKPGQAPRLLIYGAFSRATGIPDRFSGSGSGTDFTLTISRLEPEDFAVYYCQQYGSSPWTFGQGTKVEIKRTVAAPSVFIFPPSDEQLKSGTASVVCLLNNFYPREAKVQWKVDNALQSGNSQESVTEQDSKDSTYSLSSTLTLSKADYEKHKVYACEVTHQGLSSPVTKSFNRGEC

SEQ ID NO: 128 - DNA, 645 bp, Homo
gagatcgtgctgactcagagccccggcactctgtctctgagccccggcgaaagggccacactgagctgtagggctagccagagcgtgggcagcagctatctggcttggtaccagcagaagcccggccaagcccctagactgctgatctacggcgccttctctagggctactggcatcccagataggtttagcggcagcggatccggcacagacttcactctgacaatctctaggctggagccagaagacttcgccgtgtactattgccagcagtacggcagcagcccatggactttcggccaaggcacaaaggtcgagatcaagagaaccgtcgccgctcccagcgtcttcatcttcccccccagcgatgagcagctgaagagcggaaccgccagcgtggtgtgcctgctgaacaacttctaccccagggaggccaaggtgcaatggaaggtggacaacgccctacagagcggcaactcccaggagagcgtgaccgagcaggacagcaaggatagcacctacagcctgagcagcaccctcaccctgagcaaggccgactacgagaagcacaaggtgtacgcctgcgaggtgacccatcagggcctgagcagccctgtgaccaagagcttcaacaggggcgagtgc

SEQ ID NO: 129 - protein, 214 aa, Homo
DIQMTQSPSSLSASVGDRVTITCRASQDISNYLSWYQQKPGKTIKLLIYYTSRLHSGVPSRFSGSGSGTDYTFTISSLQPEDIATYFCQQGKTLPYTFGQGTKVEIKRTVAAPSVFIFPPSDEQLKSGTASVVCLLNNFYPREAKVQWKVDNALQSGNSQESVTEQDSKDSTYSLSSTLTLSKADYEKHKVYACEVTHQGLSSPVTKSFNRGEC

SEQ ID NO: 130 - DNA, 642 bp, Homo
gacatccagatgacccagtccccttcctccctgtccgcttccgtgggcgacagggtgaccatcacctgcagggccagccaggacatctccaactacctgtcctggtaccagcagaagcccggcaagaccatcaagctgctgatctactacacctccaggctgcacagcggcgtgcctagcaggttctccggttctggctccggcaccgactacaccttcaccatcagctccctgcagcccgaggacatcgccacctacttctgccagcagggcaagaccctgccctacaccttcggccagggcaccaaggtggagatcaagcgcactgtggctgcccccagtgttttcatatttccccccagtgatgagcaactgaagtccggcacagcctctgttgtatgtctgctgaataatttttatccacgggaggccaaggtgcagtggaaggtggacaatgccctgcagtctgggaactctcaagagagtgtgacagagcaggacagtaaagacagcacctatagcctcagcagcaccctgaccctgtctaaagccgactatgaaaaacacaaagtgtatgcctgcgaagtgacccatcaggggctcagctctcccgttaccaagagctttaaccgaggcgaatgt

SEQ ID NO: 131 - protein, 676 aa, Homo
EVKLVESGGGLVQPGGSLRLSCAASGFAFSSYDMSWVRQAPGKRLEWVATISGGGRYTYYPDTVKGRFTISRDNAKNSHYLQMNSLRAEDTAVYFCASPYGGYFDVWGQGTLVTVSSASTKGPSVFPLAPCSRSTSESTAALGCLVKDYFPEPVTVSWNSGALTSGVHTFPAVLQSSGLYSLSSVVTVPSSSLGTKTYTCNVDHKPSNTKVDKRVGGGGSGGGGSGGGGSQVQLKQSGPGLVQPSQSLSITCTVSGFSLTNYGVHWVRQSPGKGLEWLGVIWSGGNTDYNTPFTSRLSINKDNSKSQVFFKMNSLQSNDTAIYYCARALTYYDYEFAYWGQGTLVTVSAASTKGPSVFPLAPCSRSTSESTAALGCLVKDYFPEPVTVSWNSGALTSGVHTFPAVLQSSGLYSLSSVVTVPSSSLGTKTYTCNVDHKPSNTKVDKRVESKYGPPCPPCPAPEFLGGPSVFLFPPKPKDTLMISRTPEVTCVVVDVSQEDPEVQFNWYVDGVEVHNAKTKPREEQFNSTYRVVSVLTVLHQDWLNGKEYKCKVSNKGLPSSIEKTISKAKGQPREPQVYTLPPSQEEMTKNQVSLTCLVKGFYPSDIAVEWESNGQPENNYKTTPPVLDSDGSFFLYSRLTVDKSRWQEGNVFSCSVMHEALHNHYTQKSLSLSLGK

SEQ ID NO: 132 - DNA, 2028 bp, Homo
gaggtcaagctggtggaaagcggcggcggcctggtgcagcctggaggatccctgcggctgagctgcgctgcctccggcttcgctttcagctcctatgacatgtcctgggtgaggcaggcccctggaaagaggctggagtgggtggctaccatctccggaggcggaaggtacacctactaccccgacacagtgaagggaaggttcaccatcagccgggataacgccaaaaacagccactatctccagatgaactccctgagggccgaagatacagccgtgtatttctgtgcctccccctacggaggctattttgacgtgtggggacagggcaccctggtgaccgtctcctccgcaagtaccaagggacctagtgttttccctcttgcaccttgctccaggtcaacatcagagtccacagctgctcttggatgtctcgttaaggactacttcccagagccagttaccgtatcctggaactccggagctttgacaagcggcgttcatacattcccagctgtgttgcagagttctgggttgtacagtttgagctcagtggtgaccgtgccttcatcttctttgggcactaagacctacacctgcaacgtggatcacaagccaagcaacaccaaggtggataagagggtgggtggaggcggttcaggcggaggtggcagcggaggtggcgggagtcaggtgcagctgaagcagtccggacctggcctggtgcagccttcccagtccctgtccatcacctgcaccgtgtccggcttttccctgaccaactacggcgtgcactgggtgaggcagtcccctggcaagggcctggaatggctgggcgtgatctggtccggcggcaacaccgactacaacacccccttcacctcccggctgtccatcaacaaggacaacagcaagtcccaggtgttcttcaagatgaactccctgcagagcaacgacaccgccatctactactgcgccagagccctgacctattacgactacgagttcgcctactggggccagggcacactggtgaccgtgtccgccgcctccaccaagggcccatcggtcttccccctggcaccctgctccaggagcacctctgagtccacagcggccctgggctgcctggtcaaggactacttccccgaaccggtgacggtgtcgtggaactcaggcgccctgaccagcggcgtgcacaccttcccggctgtcctacagtcctcaggactctactccctcagcagcgtggtgaccgtgccctccagcagcttgggcaccaagacatatacctgtaatgtggatcacaagccttccaatacaaaagtggacaagagagttgagtccaagtacggcccaccatgtcctccatgtccagcccctgaatttttgggcgggccttctgtctttctgtttcctcctaaacctaaagataccctgatgatcagccgcacacccgaagtcacttgtgtggtcgtggatgtgtctcaggaagatcccgaagtgcagtttaactggtatgtcgatggcgtggaagtgcataatgccaaaactaagccccgcgaagaacagttcaacagcacttatcgggtcgtgtctgtgctcacagtcctccatcaggattggctgaatgggaaagaatataagtgcaaggtgagcaataagggcctccccagcagcatcgagaagactattagcaaagccaaagggcagccacgggaaccccaggtgtacactctgcccccctctcaggaggagatgactaaaaatcaggtctctctgacttgtctggtgaaagggttttatcccagcgacattgccgtggagtgggagtctaatggccagcccgagaataattataagacaactccccccgtcctggactctgacggcagctttttcctgtattctcggctgacagtggacaaaagtcgctggcaggagggcaatgtctttagttgcagtgtcatgcatgaggccctgcacaatcactatacacagaaaagcctgtctctgagtctgggcaaa

SEQ ID NO: 133 - protein, 676 aa, Homo
EVKLVESGGGLVQPGGSLRLSCAASGFAFSSYDMSWVRQAPGKRLEWVATISGGGRYTYYPDTVKGRFTISRDNAKNSHYLQMNSLRAEDTAVYFCASPYGGYFDVWGQGTLVTVSSASTKGPSVFPLAPCSRSTSESTAALGCLVKDYFPEPVTVSWNSGALTSGVHTFPAVLQSSGLYSLSSVVTVPSSSLGTKTYTCNVDHKPSNTKVDKRVGGGGSGGGGSGGGGSEVQLVESGGGLVQPGGSLRLSCAASGFTFTDYTMDWVRQAPGKGLEWVADVNPNSGGSIYNQRFKGRFTLSVDRSKNTLYLQMNSLRAEDTAVYYCARNLGPSFYFDYWGQGTLVTVSSASTKGPSVFPLAPCSRSTSESTAALGCLVKDYFPEPVTVSWNSGALTSGVHTFPAVLQSSGLYSLSSVVTVPSSSLGTKTYTCNVDHKPSNTKVDKRVESKYGPPCPPCPAPEFLGGPSVFLFPPKPKDTLMISRTPEVTCVVVDVSQEDPEVQFNWYVDGVEVHNAKTKPREEQFNSTYRVVSVLTVLHQDWLNGKEYKCKVSNKGLPSSIEKTISKAKGQPREPQVYTLPPSQEEMTKNQVSLTCLVKGFYPSDIAVEWESNGQPENNYKTTPPVLDSDGSFFLYSRLTVDKSRWQEGNVFSCSVMHEALHNHYTQKSLSLSLGK

SEQ ID NO: 134 - DNA, 2028 bp, Homo
gaggtcaagctggtggaaagcggcggcggcctggtgcagcctggaggatccctgcggctgagctgcgctgcctccggcttcgctttcagctcctatgacatgtcctgggtgaggcaggcccctggaaagaggctggagtgggtggctaccatctccggaggcggaaggtacacctactaccccgacacagtgaagggaaggttcaccatcagccgggataacgccaaaaacagccactatctccagatgaactccctgagggccgaagatacagccgtgtatttctgtgcctccccctacggaggctattttgacgtgtggggacagggcaccctggtgaccgtctcctccgcaagtaccaagggacctagtgttttccctcttgcaccttgctccaggtcaacatcagagtccacagctgctcttggatgtctcgttaaggactacttcccagagccagttaccgtatcctggaactccggagctttgacaagcggcgttcatacattcccagctgtgttgcagagttctgggttgtacagtttgagctcagtggtgaccgtgccttcatcttctttgggcactaagacctacacctgcaacgtggatcacaagccaagcaacaccaaggtggataagagggtgggtggaggcggttcaggcggaggtggcagcggaggtggcgggagtgaagtgcagctggtggagtctggaggcggactggtgcagcctggaggctctctgagactgtcttgtgctgcttctggctttacctttaccgattataccatggattgggtgagacaggcccctggaaagggactggagtgggtggctgatgtgaaccctaactctggaggatctatctataatcagaggtttaagggcagattcaccctgtctgtggatagatctaagaatacactgtatctgcagatgaactctctgagagctgaagatacagctgtgtattactgcgctagaaatctgggcccttccttttactttgattactggggccagggaacactggtgaccgtgtcttctgcctccaccaagggcccatcggtcttccccctggcaccctgctccaggagcacctctgagtccacagcggccctgggctgcctggtcaaggactacttccccgaaccggtgacggtgtcgtggaactcaggcgccctgaccagcggcgtgcacaccttcccggctgtcctacagtcctcaggactctactccctcagcagcgtggtgaccgtgccctccagcagcttgggcaccaagacatatacctgtaatgtggatcacaagccttccaatacaaaagtggacaagagagttgagtccaagtacggcccaccatgtcctccatgtccagcccctgaatttttgggcgggccttctgtctttctgtttcctcctaaacctaaagataccctgatgatcagccgcacacccgaagtcacttgtgtggtcgtggatgtgtctcaggaagatcccgaagtgcagtttaactggtatgtcgatggcgtggaagtgcataatgccaaaactaagccccgcgaagaacagttcaacagcacttatcgggtcgtgtctgtgctcacagtcctccatcaggattggctgaatgggaaagaatataagtgcaaggtgagcaataagggcctccccagcagcatcgagaagactattagcaaagccaaagggcagccacgggaaccccaggtgtacactctgcccccctctcaggaggagatgactaaaaatcaggtctctctgacttgtctggtgaaagggttttatcccagcgacattgccgtggagtgggagtctaatggccagcccgagaataattataagacaactccccccgtcctggactctgacggcagctttttcctgtattctcggctgacagtggacaaaagtcgctggcaggagggcaatgtctttagttgcagtgtcatgcatgaggccctgcacaatcactatacacagaaaagcctgtctctgagtctgggcaaa

SEQ ID NO: 135 - protein, 678 aa, Homo
EVKLVESGGGLVQPGGSLRLSCAASGFAFSSYDMSWVRQAPGKRLEWVATISGGGRYTYYPDTVKGRFTISRDNAKNSHYLQMNSLRAEDTAVYFCASPYGGYFDVWGQGTLVTVSSASTKGPSVFPLAPCSRSTSESTAALGCLVKDYFPEPVTVSWNSGALTSGVHTFPAVLQSSGLYSLSSVVTVPSSSLGTKTYTCNVDHKPSNTKVDKRVGGGGSGGGGSGGGGSQVQLVESGGGVVQPGRSLRLSCAASGFTFSSYTMHWVRQAPGKGLEWVTFISYDGNNKYYADSVKGRFTISRDNSKNTLYLQMNSLRAEDTAIYYCARTGWLGPFDYWGQGTLVTVSSASTKGPSVFPLAPSSKSTSGGTAALGCLVKDYFPEPVTVSWNSGALTSGVHTFPAVLQSSGLYSLSSVVTVPSSSLGTQTYICNVNHKPSNTKVDKKVEPKSCDKTHTCPPCPAPELLGGPSVFLFPPKPKDTLMISRTPEVTCVVVDVSHEDPEVKFNWYVDGVEVHNAKTKPREEQYNSTYRVVSVLTVLHQDWLNGKEYKCKVSNKALPAPIEKTISKAKGQPREPQVYTLPPSREEMTKNQVSLTCLVKGFYPSDIAVEWESNGQPENNYKTTPPVLDSDGSFFLYSKLTVDKSRWQQGNVFSCSVMHEALHNHYTQKSLSLSPGK

SEQ ID NO: 136 - DNA, 2034 bp, Homo
gaggtcaagctggtggaaagcggcggcggcctggtgcagcctggaggatccctgcggctgagctgcgctgcctccggcttcgctttcagctcctatgacatgtcctgggtgaggcaggcccctggaaagaggctggagtgggtggctaccatctccggaggcggaaggtacacctactaccccgacacagtgaagggaaggttcaccatcagccgggataacgccaaaaacagccactatctccagatgaactccctgagggccgaagatacagccgtgtatttctgtgcctccccctacggaggctattttgacgtgtggggacagggcaccctggtgaccgtctcctccgcaagtaccaagggacctagtgttttccctcttgcaccttgctccaggtcaacatcagagtccacagctgctcttggatgtctcgttaaggactacttcccagagccagttaccgtatcctggaactccggagctttgacaagcggcgttcatacattcccagctgtgttgcagagttctgggttgtacagtttgagctcagtggtgaccgtgccttcatcttctttgggcactaagacctacacctgcaacgtggatcacaagccaagcaacaccaaggtggataagagggtgggtggaggcggttcaggcggaggtggcagcggaggtggcgggagtcaagtgcagctggtcgaaagcggcggaggagtcgtccagcccggcagatctctgagactgagctgtgctgcctccggcttcacattcagctcctacactatgcactgggtgaggcaagcccccggcaagggactggagtgggtgactttcatcagctacgacggcaacaacaagtactacgccgacagcgtgaagggaaggttcactatctctagggacaacagcaagaacactctgtatctgcagatgaactctctgagggccgaggatactgccatctactactgcgctaggactggctggctgggccctttcgattactggggccaaggcactctggtcactgtgagcagcgcgagcaccaagggaccttccgtgtttcccctcgcccccagctccaaaagcaccagcggcggaacagctgctctcggctgtctcgtcaaggattacttccccgagcccgtgaccgtgagctggaacagcggagccctgacaagcggcgtccacaccttccctgctgtcctacagtcctccggactgtacagcctgagcagcgtggtgacagtccctagcagctccctgggcacccagacatatatttgcaacgtgaatcacaagcccagcaacaccaaggtcgataagaaggtggagcctaagtcctgcgacaagacccacacatgtcccccctgtcccgctcctgaactgctgggaggcccttccgtgttcctgttcccccctaagcccaaggacaccctgatgatttccaggacacccgaggtgacctgtgtggtggtggacgtcagccacgaggaccccgaggtgaaattcaactggtacgtcgatggcgtggaggtgcacaacgctaagaccaagcccagggaggagcagtacaattccacctacagggtggtgtccgtgctgaccgtcctccatcaggactggctgaacggcaaagagtataagtgcaaggtgagcaacaaggccctccctgctcccatcgagaagaccatcagcaaagccaagggccagcccagggaacctcaagtctataccctgcctcccagcagggaggagatgaccaagaaccaagtgagcctcacatgcctcgtcaagggcttctatccttccgatattgccgtcgagtgggagtccaacggacagcccgagaacaactacaagacaacaccccccgtgctcgattccgatggcagcttcttcctgtactccaagctgaccgtggacaagtccagatggcaacaaggcaacgtcttcagttgcagcgtcatgcatgaggccctccacaaccactacacccagaaaagcctgtctctgagtcctggcaaa

SEQ ID NO: 137 - protein, 678 aa, Homo
QVQLVESGGGVVQPGRSLRLSCAASGFTFSSYTMHWVRQAPGKGLEWVTFISYDGNNKYYADSVKGRFTISRDNSKNTLYLQMNSLRAEDTAIYYCARTGWLGPFDYWGQGTLVTVSSASTKGPSVFPLAPCSRSTSESTAALGCLVKDYFPEPVTVSWNSGALTSGVHTFPAVLQSSGLYSLSSVVTVPSSSLGTKTYTCNVDHKPSNTKVDKRVGGGGSGGGGSGGGGSEVKLVESGGGLVQPGGSLRLSCAASGFAFSSYDMSWVRQAPGKRLEWVATISGGGRYTYYPDTVKGRFTISRDNAKNSHYLQMNSLRAEDTAVYFCASPYGGYFDVWGQGTLVTVSSASTKGPSVFPLAPSSKSTSGGTAALGCLVKDYFPEPVTVSWNSGALTSGVHTFPAVLQSSGLYSLSSVVTVPSSSLGTQTYICNVNHKPSNTKVDKKVEPKSCDKTHTCPPCPAPELLGGPSVFLFPPKPKDTLMISRTPEVTCVVVDVSHEDPEVKFNWYVDGVEVHNAKTKPREEQYNSTYRVVSVLTVLHQDWLNGKEYKCKVSNKALPAPIEKTISKAKGQPREPQVYTLPPSREEMTKNQVSLTCLVKGFYPSDIAVEWESNGQPENNYKTTPPVLDSDGSFFLYSKLTVDKSRWQQGNVFSCSVMHEALHNHYTQKSLSLSPGK

SEQ ID NO: 138 - DNA, 2034 bp, Homo
caagtgcagctggtcgaaagcggcggaggagtcgtccagcccggcagatctctgagactgagctgtgctgcctccggcttcacattcagctcctacactatgcactgggtgaggcaagcccccggcaagggactggagtgggtgactttcatcagctacgacggcaacaacaagtactacgccgacagcgtgaagggaaggttcactatctctagggacaacagcaagaacactctgtatctgcagatgaactctctgagggccgaggatactgccatctactactgcgctaggactggctggctgggccctttcgattactggggccaaggcactctggtcactgtgagcagcgcaagtaccaagggacctagtgttttccctcttgcaccttgctccaggtcaacatcagagtccacagctgctcttggatgtctcgttaaggactacttcccagagccagttaccgtatcctggaactccggagctttgacaagcggcgttcatacattcccagctgtgttgcagagttctgggttgtacagtttgagctcagtggtgaccgtgccttcatcttctttgggcactaagacctacacctgcaacgtggatcacaagccaagcaacaccaaggtggataagagggtgggtggaggcggttcaggcggaggtggcagcggaggtggcgggagtgaggtcaagctggtggaaagcggcggcggcctggtgcagcctggaggatccctgcggctgagctgcgctgcctccggcttcgctttcagctcctatgacatgtcctgggtgaggcaggcccctggaaagaggctggagtgggtggctaccatctccggaggcggaaggtacacctactaccccgacacagtgaagggaaggttcaccatcagccgggataacgccaaaaacagccactatctccagatgaactccctgagggccgaagatacagccgtgtatttctgtgcctccccctacggaggctattttgacgtgtggggacagggcaccctggtgaccgtctcctccgcgagcaccaagggaccttccgtgtttcccctcgcccccagctccaaaagcaccagcggcggaacagctgctctcggctgtctcgtcaaggattacttccccgagcccgtgaccgtgagctggaacagcggagccctgacaagcggcgtccacaccttccctgctgtcctacagtcctccggactgtacagcctgagcagcgtggtgacagtccctagcagctccctgggcacccagacatatatttgcaacgtgaatcacaagcccagcaacaccaaggtcgataagaaggtggagcctaagtcctgcgacaagacccacacatgtcccccctgtcccgctcctgaactgctgggaggcccttccgtgttcctgttcccccctaagcccaaggacaccctgatgatttccaggacacccgaggtgacctgtgtggtggtggacgtcagccacgaggaccccgaggtgaaattcaactggtacgtcgatggcgtggaggtgcacaacgctaagaccaagcccagggaggagcagtacaattccacctacagggtggtgtccgtgctgaccgtcctccatcaggactggctgaacggcaaagagtataagtgcaaggtgagcaacaaggccctccctgctcccatcgagaagaccatcagcaaagccaagggccagcccagggaacctcaagtctataccctgcctcccagcagggaggagatgaccaagaaccaagtgagcctcacatgcctcgtcaagggcttctatccttccgatattgccgtcgagtgggagtccaacggacagcccgagaacaactacaagacaacaccccccgtgctcgattccgatggcagcttcttcctgtactccaagctgaccgtggacaagtccagatggcaacaaggcaacgtcttcagttgcagcgtcatgcatgaggccctccacaaccactacacccagaaaagcctgtctctgagtcctggcaaa

SEQ ID NO: 139 - protein, 675 aa, Homo
EVKLVESGGGLVQPGGSLRLSCAASGFAFSSYDMSWVRQAPGKRLEWVATISGGGRYTYYPDTVKGRFTISRDNAKNSHYLQMNSLRAEDTAVYFCASPYGGYFDVWGQGTLVTVSSASTKGPSVFPLAPCSRSTSESTAALGCLVKDYFPEPVTVSWNSGALTSGVHTFPAVLQSSGLYSLSSVVTVPSSSLGTKTYTCNVDHKPSNTKVDKRVGGGGSGGGGSGGGGSQVQLVESGGGVVQPGRSLRLSCAASGFTFSSYTMHWVRQAPGKGLEWVTFISYDGNNKYYADSVKGRFTISRDNSKNTLYLQMNSLRAEDTAIYYCARTGWLGPFDYWGQGTLVTVSSASTKGPSVFPLAPCSRSTSESTAALGCLVKDYFPEPVTVSWNSGALTSGVHTFPAVLQSSGLYSLSSVVTVPSSSLGTKTYTCNVDHKPSNTKVDKRVESKYGPPCPPCPAPEFLGGPSVFLFPPKPKDTLMISRTPEVTCVVVDVSQEDPEVQFNWYVDGVEVHNAKTKPREEQFNSTYRVVSVLTVLHQDWLNGKEYKCKVSNKGLPSSIEKTISKAKGQPREPQVYTLPPSQEEMTKNQVSLTCLVKGFYPSDIAVEWESNGQPENNYKTTPPVLDSDGSFFLYSRLTVDKSRWQEGNVFSCSVMHEALHNHYTQKSLSLSLGK

SEQ ID NO: 140 - DNA, 2025 bp, Homo
gaggtcaagctggtggaaagcggcggcggcctggtgcagcctggaggatccctgcggctgagctgcgctgcctccggcttcgctttcagctcctatgacatgtcctgggtgaggcaggcccctggaaagaggctggagtgggtggctaccatctccggaggcggaaggtacacctactaccccgacacagtgaagggaaggttcaccatcagccgggataacgccaaaaacagccactatctccagatgaactccctgagggccgaagatacagccgtgtatttctgtgcctccccctacggaggctattttgacgtgtggggacagggcaccctggtgaccgtctcctccgcaagtaccaagggacctagtgttttccctcttgcaccttgctccaggtcaacatcagagtccacagctgctcttggatgtctcgttaaggactacttcccagagccagttaccgtatcctggaactccggagctttgacaagcggcgttcatacattcccagctgtgttgcagagttctgggttgtacagtttgagctcagtggtgaccgtgccttcatcttctttgggcactaagacctacacctgcaacgtggatcacaagccaagcaacaccaaggtggataagagggtgggtggaggcggttcaggcggaggtggcagcggaggtggcgggagtcaagtgcagctggtcgaaagcggcggaggagtcgtccagcccggcagatctctgagactgagctgtgctgcctccggcttcacattcagctcctacactatgcactgggtgaggcaagcccccggcaagggactggagtgggtgactttcatcagctacgacggcaacaacaagtactacgccgacagcgtgaagggaaggttcactatctctagggacaacagcaagaacactctgtatctgcagatgaactctctgagggccgaggatactgccatctactactgcgctaggactggctggctgggccctttcgattactggggccaaggcactctggtcactgtgagcagcgcctccaccaagggcccatcggtcttccccctggcaccctgctccaggagcacctctgagtccacagcggccctgggctgcctggtcaaggactacttccccgaaccggtgacggtgtcgtggaactcaggcgccctgaccagcggcgtgcacaccttcccggctgtcctacagtcctcaggactctactccctcagcagcgtggtgaccgtgccctccagcagcttgggcaccaagacatatacctgtaatgtggatcacaagccttccaatacaaaagtggacaagagagttgagtccaagtacggcccaccatgtcctccatgtccagcccctgaatttttgggcgggccttctgtctttctgtttcctcctaaacctaaagataccctgatgatcagccgcacacccgaagtcacttgtgtggtcgtggatgtgtctcaggaagatcccgaagtgcagtttaactggtatgtcgatggcgtggaagtgcataatgccaaaactaagccccgcgaagaacagttcaacagcacttatcgggtcgtgtctgtgctcacagtcctccatcaggattggctgaatgggaaagaatataagtgcaaggtgagcaataagggcctccccagcagcatcgagaagactattagcaaagccaaagggcagccacgggaaccccaggtgtacactctgcccccctctcaggaggagatgactaaaaatcaggtctctctgacttgtctggtgaaagggttttatcccagcgacattgccgtggagtgggagtctaatggccagcccgagaataattataagacaactccccccgtcctggactctgacggcagctttttcctgtattctcggctgacagtggacaaaagtcgctggcaggagggcaatgtctttagttgcagtgtcatgcatgaggccctgcacaatcactatacacagaaaagcctgtctctgagtctgggcaaa

SEQ ID NO: 141 - protein, 675 aa, Homo
QVQLVESGGGVVQPGRSLRLSCAASGFTFSSYTMHWVRQAPGKGLEWVTFISYDGNNKYYADSVKGRFTISRDNSKNTLYLQMNSLRAEDTAIYYCARTGWLGPFDYWGQGTLVTVSSASTKGPSVFPLAPCSRSTSESTAALGCLVKDYFPEPVTVSWNSGALTSGVHTFPAVLQSSGLYSLSSVVTVPSSSLGTKTYTCNVDHKPSNTKVDKRVGGGGSGGGGSGGGGSEVKLVESGGGLVQPGGSLRLSCAASGFAFSSYDMSWVRQAPGKRLEWVATISGGGRYTYYPDTVKGRFTISRDNAKNSHYLQMNSLRAEDTAVYFCASPYGGYFDVWGQGTLVTVSSASTKGPSVFPLAPCSRSTSESTAALGCLVKDYFPEPVTVSWNSGALTSGVHTFPAVLQSSGLYSLSSVVTVPSSSLGTKTYTCNVDHKPSNTKVDKRVESKYGPPCPPCPAPEFLGGPSVFLFPPKPKDTLMISRTPEVTCVVVDVSQEDPEVQFNWYVDGVEVHNAKTKPREEQFNSTYRVVSVLTVLHQDWLNGKEYKCKVSNKGLPSSIEKTISKAKGQPREPQVYTLPPSQEEMTKNQVSLTCLVKGFYPSDIAVEWESNGQPENNYKTTPPVLDSDGSFFLYSRLTVDKSRWQEGNVFSCSVMHEALHNHYTQKSLSLSLGK

SEQ ID NO: 142 - DNA, 2025 bp, Homo
caagtgcagctggtcgaaagcggcggaggagtcgtccagcccggcagatctctgagactgagctgtgctgcctccggcttcacattcagctcctacactatgcactgggtgaggcaagcccccggcaagggactggagtgggtgactttcatcagctacgacggcaacaacaagtactacgccgacagcgtgaagggaaggttcactatctctagggacaacagcaagaacactctgtatctgcagatgaactctctgagggccgaggatactgccatctactactgcgctaggactggctggctgggccctttcgattactggggccaaggcactctggtcactgtgagcagcgcaagtaccaagggacctagtgttttccctcttgcaccttgctccaggtcaacatcagagtccacagctgctcttggatgtctcgttaaggactacttcccagagccagttaccgtatcctggaactccggagctttgacaagcggcgttcatacattcccagctgtgttgcagagttctgggttgtacagtttgagctcagtggtgaccgtgccttcatcttctttgggcactaagacctacacctgcaacgtggatcacaagccaagcaacaccaaggtggataagagggtgggtggaggcggttcaggcggaggtggcagcggaggtggcgggagtgaggtcaagctggtggaaagcggcggcggcctggtgcagcctggaggatccctgcggctgagctgcgctgcctccggcttcgctttcagctcctatgacatgtcctgggtgaggcaggcccctggaaagaggctggagtgggtggctaccatctccggaggcggaaggtacacctactaccccgacacagtgaagggaaggttcaccatcagccgggataacgccaaaaacagccactatctccagatgaactccctgagggccgaagatacagccgtgtatttctgtgcctccccctacggaggctattttgacgtgtggggacagggcaccctggtgaccgtctcctccgcctccaccaagggcccatcggtcttccccctggcaccctgctccaggagcacctctgagtccacagcggccctgggctgcctggtcaaggactacttccccgaaccggtgacggtgtcgtggaactcaggcgccctgaccagcggcgtgcacaccttcccggctgtcctacagtcctcaggactctactccctcagcagcgtggtgaccgtgccctccagcagcttgggcaccaagacatatacctgtaatgtggatcacaagccttccaatacaaaagtggacaagagagttgagtccaagtacggcccaccatgtcctccatgtccagcccctgaatttttgggcgggccttctgtctttctgtttcctcctaaacctaaagataccctgatgatcagccgcacacccgaagtcacttgtgtggtcgtggatgtgtctcaggaagatcccgaagtgcagtttaactggtatgtcgatggcgtggaagtgcataatgccaaaactaagccccgcgaagaacagttcaacagcacttatcgggtcgtgtctgtgctcacagtcctccatcaggattggctgaatgggaaagaatataagtgcaaggtgagcaataagggcctccccagcagcatcgagaagactattagcaaagccaaagggcagccacgggaaccccaggtgtacactctgcccccctctcaggaggagatgactaaaaatcaggtctctctgacttgtctggtgaaagggttttatcccagcgacattgccgtggagtgggagtctaatggccagcccgagaataattataagacaactccccccgtcctggactctgacggcagctttttcctgtattctcggctgacagtggacaaaagtcgctggcaggagggcaatgtctttagttgcagtgtcatgcatgaggccctgcacaatcactatacacagaaaagcctgtctctgagtctgggcaaa

SEQ ID NO: 143 - protein, 673 aa, Homo
EVKLVESGGGLVQPGGSLRLSCAASGFAFSSYDMSWVRQAPGKRLEWVATISGGGRYTYYPDTVKGRFTISRDNAKNSHYLQMNSLRAEDTAVYFCASPYGGYFDVWGQGTLVTVSSASTKGPSVFPLAPCSRSTSESTAALGCLVKDYFPEPVTVSWNSGALTSGVHTFPAVLQSSGLYSLSSVVTVPSSSLGTKTYTCNVDHKPSNTKVDKRVGGGGSGGGGSGGGGSEVQLVESGGGLVKPGGSLRLSCAASGFTFSDDYMAWFRQAPGKRLEWVASISHGGDYIYYADNLKGRFTISRDNAKNSLYLQMNSLRAEDTAVYFCSRDRRSIDYWGQGTLVTVSSASTKGPSVFPLAPCSRSTSESTAALGCLVKDYFPEPVTVSWNSGALTSGVHTFPAVLQSSGLYSLSSVVTVPSSSLGTKTYTCNVDHKPSNTKVDKRVESKYGPPCPPCPAPEFLGGPSVFLFPPKPKDTLMISRTPEVTCVVVDVSQEDPEVQFNWYVDGVEVHNAKTKPREEQFNSTYRVVSVLTVLHQDWLNGKEYKCKVSNKGLPSSIEKTISKAKGQPREPQVYTLPPSQEEMTKNQVSLTCLVKGFYPSDIAVEWESNGQPENNYKTTPPVLDSDGSFFLYSRLTVDKSRWQEGNVFSCSVMHEALHNHYTQKSLSLSLGK

SEQ ID NO: 144 - DNA, 2019 bp, Homo
gaggtcaagctggtggaaagcggcggcggcctggtgcagcctggaggatccctgcggctgagctgcgctgcctccggcttcgctttcagctcctatgacatgtcctgggtgaggcaggcccctggaaagaggctggagtgggtggctaccatctccggaggcggaaggtacacctactaccccgacacagtgaagggaaggttcaccatcagccgggataacgccaaaaacagccactatctccagatgaactccctgagggccgaagatacagccgtgtatttctgtgcctccccctacggaggctattttgacgtgtggggacagggcaccctggtgaccgtctcctccgcaagtaccaagggacctagtgttttccctcttgcaccttgctccaggtcaacatcagagtccacagctgctcttggatgtctcgttaaggactacttcccagagccagttaccgtatcctggaactccggagctttgacaagcggcgttcatacattcccagctgtgttgcagagttctgggttgtacagtttgagctcagtggtgaccgtgccttcatcttctttgggcactaagacctacacctgcaacgtggatcacaagccaagcaacaccaaggtggataagagggtgggtggaggcggttcaggcggaggtggcagcggaggtggcgggagtgaagtgcagctggtggagtccggaggcggactggtgaagcctggaggctccctgaggctgtcctgtgccgcttccggcttcaccttctccgacgactacatggcctggttcaggcaggcccctggaaagaggctggagtgggtggcttccatctcccacggcggcgactacatctactacgccgacaacctgaagggcaggttcaccatctccagggacaacgccaagaactccctgtacctgcagatgaactccctgagggccgaggacaccgccgtgtacttctgctccagggacaggaggtccatcgactattggggccagggcaccctggtgacagtgtcctccgcctccaccaagggcccatcggtcttccccctggcaccctgctccaggagcacctctgagtccacagcggccctgggctgcctggtcaaggactacttccccgaaccggtgacggtgtcgtggaactcaggcgccctgaccagcggcgtgcacaccttcccggctgtcctacagtcctcaggactctactccctcagcagcgtggtgaccgtgccctccagcagcttgggcaccaagacatatacctgtaatgtggatcacaagccttccaatacaaaagtggacaagagagttgagtccaagtacggcccaccatgtcctccatgtccagcccctgaatttttgggcgggccttctgtctttctgtttcctcctaaacctaaagataccctgatgatcagccgcacacccgaagtcacttgtgtggtcgtggatgtgtctcaggaagatcccgaagtgcagtttaactggtatgtcgatggcgtggaagtgcataatgccaaaactaagccccgcgaagaacagttcaacagcacttatcgggtcgtgtctgtgctcacagtcctccatcaggattggctgaatgggaaagaatataagtgcaaggtgagcaataagggcctccccagcagcatcgagaagactattagcaaagccaaagggcagccacgggaaccccaggtgtacactctgcccccctctcaggaggagatgactaaaaatcaggtctctctgacttgtctggtgaaagggttttatcccagcgacattgccgtggagtgggagtctaatggccagcccgagaataattataagacaactccccccgtcctggactctgacggcagctttttcctgtattctcggctgacagtggacaaaagtcgctggcaggagggcaatgtctttagttgcagtgtcatgcatgaggccctgcacaatcactatacacagaaaagcctgtctctgagtctgggcaaa

SEQ ID NO: 145 - protein, 673 aa, Homo
EVQLVESGGGLVKPGGSLRLSCAASGFTFSDDYMAWFRQAPGKRLEWVASISHGGDYIYYADNLKGRFTISRDNAKNSLYLQMNSLRAEDTAVYFCSRDRRSIDYWGQGTLVTVSSASTKGPSVFPLAPCSRSTSESTAALGCLVKDYFPEPVTVSWNSGALTSGVHTFPAVLQSSGLYSLSSVVTVPSSSLGTKTYTCNVDHKPSNTKVDKRVGGGGSGGGGSGGGGSEVKLVESGGGLVQPGGSLRLSCAASGFAFSSYDMSWVRQAPGKRLEWVATISGGGRYTYYPDTVKGRFTISRDNAKNSHYLQMNSLRAEDTAVYFCASPYGGYFDVWGQGTLVTVSSASTKGPSVFPLAPCSRSTSESTAALGCLVKDYFPEPVTVSWNSGALTSGVHTFPAVLQSSGLYSLSSVVTVPSSSLGTKTYTCNVDHKPSNTKVDKRVESKYGPPCPPCPAPEFLGGPSVFLFPPKPKDTLMISRTPEVTCVVVDVSQEDPEVQFNWYVDGVEVHNAKTKPREEQFNSTYRVVSVLTVLHQDWLNGKEYKCKVSNKGLPSSIEKTISKAKGQPREPQVYTLPPSQEEMTKNQVSLTCLVKGFYPSDIAVEWESNGQPENNYKTTPPVLDSDGSFFLYSRLTVDKSRWQEGNVFSCSVMHEALHNHYTQKSLSLSLGK

SEQ ID NO: 146 - DNA, 2019 bp, Homo
gaagtgcagctggtggagtccggaggcggactggtgaagcctggaggctccctgaggctgtcctgtgccgcttccggcttcaccttctccgacgactacatggcctggttcaggcaggcccctggaaagaggctggagtgggtggcttccatctcccacggcggcgactacatctactacgccgacaacctgaagggcaggttcaccatctccagggacaacgccaagaactccctgtacctgcagatgaactccctgagggccgaggacaccgccgtgtacttctgctccagggacaggaggtccatcgactattggggccagggcaccctggtgacagtgtcctccgcaagtaccaagggacctagtgttttccctcttgcaccttgctccaggtcaacatcagagtccacagctgctcttggatgtctcgttaaggactacttcccagagccagttaccgtatcctggaactccggagctttgacaagcggcgttcatacattcccagctgtgttgcagagttctgggttgtacagtttgagctcagtggtgaccgtgccttcatcttctttgggcactaagacctacacctgcaacgtggatcacaagccaagcaacaccaaggtggataagagggtgggtggaggcggttcaggcggaggtggcagcggaggtggcgggagtgaggtcaagctggtggaaagcggcggcggcctggtgcagcctggaggatccctgcggctgagctgcgctgcctccggcttcgctttcagctcctatgacatgtcctgggtgaggcaggcccctggaaagaggctggagtgggtggctaccatctccggaggcggaaggtacacctactaccccgacacagtgaagggaaggttcaccatcagccgggataacgccaaaaacagccactatctccagatgaactccctgagggccgaagatacagccgtgtatttctgtgcctccccctacggaggctattttgacgtgtggggacagggcaccctggtgaccgtctcctccgcctccaccaagggcccatcggtcttccccctggcaccctgctccaggagcacctctgagtccacagcggccctgggctgcctggtcaaggactacttccccgaaccggtgacggtgtcgtggaactcaggcgccctgaccagcggcgtgcacaccttcccggctgtcctacagtcctcaggactctactccctcagcagcgtggtgaccgtgccctccagcagcttgggcaccaagacatatacctgtaatgtggatcacaagccttccaatacaaaagtggacaagagagttgagtccaagtacggcccaccatgtcctccatgtccagcccctgaatttttgggcgggccttctgtctttctgtttcctcctaaacctaaagataccctgatgatcagccgcacacccgaagtcacttgtgtggtcgtggatgtgtctcaggaagatcccgaagtgcagtttaactggtatgtcgatggcgtggaagtgcataatgccaaaactaagccccgcgaagaacagttcaacagcacttatcgggtcgtgtctgtgctcacagtcctccatcaggattggctgaatgggaaagaatataagtgcaaggtgagcaataagggcctccccagcagcatcgagaagactattagcaaagccaaagggcagccacgggaaccccaggtgtacactctgcccccctctcaggaggagatgactaaaaatcaggtctctctgacttgtctggtgaaagggttttatcccagcgacattgccgtggagtgggagtctaatggccagcccgagaataattataagacaactccccccgtcctggactctgacggcagctttttcctgtattctcggctgacagtggacaaaagtcgctggcaggagggcaatgtctttagttgcagtgtcatgcatgaggccctgcacaatcactatacacagaaaagcctgtctctgagtctgggcaaa

SEQ ID NO: 147 - protein, 330 aa, Homo
ASTKGPSVFPLAPSSKSTSGGTAALGCLVKDYFPEPVTVSWNSGALTSGVHTFPAVLQSSGLYSLSSVVTVPSSSLGTQTYICNVNHKPSNTKVDKKVEPKSCDKTHTCPPCPAPELLGGPSVFLFPPKPKDTLMISRTPEVTCVVVDVSHEDPEVKFNWYVDGVEVHNAKTKPREEQYNSTYRVVSVLTVLHQDWLNGKEYKCKVSNKALPAPIEKTISKAKGQPREPQVYTLPPSREEMTKNQVSLTCLVKGFYPSDIAVEWESNGQPENNYKTTPPVLDSDGSFFLYSKLTVDKSRWQQGNVFSCSVMHEALHNHYTQKSLSLSPGK

SEQ ID NO: 148 - protein, 327 aa, Homo
ASTKGPSVFPLAPCSRSTSESTAALGCLVKDYFPEPVTVSWNSGALTSGVHTFPAVLQSSGLYSLSSVVTVPSSSLGTKTYTCNVDHKPSNTKVDKRVESKYGPPCPPCPAPEFLGGPSVFLFPPKPKDTLMISRTPEVTCVVVDVSQEDPEVQFNWYVDGVEVHNAKTKPREEQFNSTYRVVSVLTVLHQDWLNGKEYKCKVSNKGLPSSIEKTISKAKGQPREPQVYTLPPSQEEMTKNQVSLTCLVKGFYPSDIAVEWESNGQPENNYKTTPPVLDSDGSFFLYSRLTVDKSRWQEGNVFSCSVMHEALHNHYTQKSLSLSLGK

SEQ ID NO: 149 - protein, 107 aa, Homo [sequence omitted]

SEQ ID NO: 150 - protein, 15 aa, Homo
GGGGSGGGGSGGGGS

SEQ ID NO: 151 - protein, 11 aa, Homo
WGQGTLVTVSS

SEQ ID NO: 152 - protein, 10 aa, Homo
FGQGTKVEIK

SEQ ID NO: 153 - protein, 10 aa, Homo
FGGGTKVELK